European Patent Application EP 4 640 699 A2, published October 29, 2025. Title: Retinal Disorders. Applicant: Ikarovec Limited. Application WO PCT/GB2022/051536, filed June 17, 2022. The sequence listing filed with the application follows.

SEQUENCE LISTING (90 sequences)

SEQ ID NO: 1 - DNA, 508 bp, synthetic construct
  misc_feature 1..508: note = cytomegalovirus (CMV) promoter
  source 1..508: mol_type = other DNA
cgttacataacttacggtaaatggcccgcctggctgaccgcccaacgacccccgcccattgacgtcaataatgacgtatgttcccatagtaacgccaatagggactttccattgacgtcaatgggtggagtatttacggtaaactgcccacttggcagtacatcaagtgtatcatatgccaagtacgccccctattgacgtcaatgacggtaaatggcccgcctggcattatgcccagtacatgaccttatgggactttcctacttggcagtacatctacgtattagtcatcgctattaccatggtgatgcggttttggcagtacatcaatgggcgtggatagcggtttgactcacggggatttccaagtctccaccccattgacgtcaatgggagtttgttttggcaccaaaatcaacgggactttccaaaatgtcgtaacaactccgccccattgacgcaaatgggcggtaggcgtgtacggtgggaggtctatataagcagagct

SEQ ID NO: 2 - DNA, 60 bp, synthetic construct
  misc_feature 1..60: note = Truncated form of the CMV promoter
  source 1..60: mol_type = other DNA
aggtaggcgtgtacggtgggaggtctatataagcagagctggtttagtgaaccgtcagat

SEQ ID NO: 3 - DNA, 583 bp, synthetic construct
  misc_feature 1..583: note = fusion promoter of the CMV early enhancer element and the first intron of the chicken beta-actin gene (CAG)
  source 1..583: mol_type = other DNA
cgttacataacttacggtaaatggcccgcctggctgaccgcccaacgacccccgcccattgacgtcaataatgacgtatgttcccatagtaacgccaatagggactttccattgacgtcaatgggtggactatttacggtaaactgcccacttggcagtacatcaagtgtatcatatgccaagtacgccccctattgacgtcaatgacggtaaatggcccgcctggcattatgcccagtacatgaccttatgggactttcctacttggcagtacatctacgtattagtcatcgctattaccatggtcgaggtgagccccacgttctgcttcactctccccatctcccccccctccccacccccaattttgtatttatttattttttaattattttgtgcagcgatgggggcggggggggggggggggcgcgcgccaggcggggcggggcggggcgaggggcggggcggggcgaggcggagaggtgcggcggcagccaatcagagcggcgcgctccgaaagtttccttttatggcgaggcggcggcggcggcggccctataaaaagcgaagcgcgcggcgggcg

SEQ ID NO: 4 - DNA, 2039 bp, synthetic construct
  misc_feature 1..2039: note = Vitelliform macular dystrophy protein-2 (VMD2) promoter
  source 1..2039: mol_type = other DNA
aattctgtcattttactagggtgatgaaattcccaagcaacaccatccttttcagataagggcactgaggctgagagaggagctgaaacctacccggcgtcaccacacacaggtggcaaggctgggaccagaaaccaggactgttgactgcagcccggtattcattctttccatagcccacagggctgtcaaagaccccagggcctagtcagaggctcctccttcctggagagttcctggcacagaagttgaagctcagcacagccccctaacccccaactctctctgcaaggcctcaggggtcagaacactggtggagcagatcctttagcctctggattttagggccatggtagagggggtgttgccctaaattccagccctggtctcagcccaacaccctccaagaagaaattagaggggccatggccaggctgtgctagccgttgcttctgagcagattacaagaagggactaagacaaggactcctttgtggaggtcctggcttagggagtcaagtgacggcggctcagcactcacgtgggcagtgccagcctctaagagtgggcaggggcactggccacagagtcccagggagtcccaccagcctagtcgccagaccttctgtgggatcatcggacccacctggaaccccacctgtgagtacaaggtgccccaggtggactgggctggggctttgaggccttcagggttggatggccatcttgcgtatttgtgtgggatatgcacacacaggcagcacatgcgcaggtgtgtgggcacctgtgtgtctgtgcaaatgccctgaggtgggaatgagcttggtgtgcatcaggcacagccagccagtgtggctgcagcaaaacacacagggaaagaatggagggggcatcaatcactgcttcagtaaatttttattgagcgccttctacgagaacacaagaggagcttccattctgaggaggaaacaggcaggaaacaggcagatatcctgtataatttcaagtagtgataagtgctctctagaaatatcaagcaaggtgaggagacacagagcaccggtggcagtggggctctatttccaggttggatggttgggaacatcctttctaaagggaacctggagtgggaaggaaccatgcaggtatctcaggaagagcttcctccaggcaggaagatcagcaggtggaaaggccctggagccaccattcagtaaacatcatttgagcatctctaccagctaggttccattatgggaatgggaatatggtggtggacagggctgcctggtcccttccatacttctcacactagggtggttgagagagcttgggagctaacgaacaagatgggctgagaacactgcctagcccagaggacctgagcttagtgtgtagacattgctgctgttactgcctttgtcattgtattatttatttatttatttatttatttttagacagagttttgctcttcttacccaggctggagtgcaatggcgtgatctcagctcactgcaacctccacctcctgggttcaagcgattctcctgcctcagcctcctgagtagctgggattacaggcacccgcaccacgcctggataatttttttgtatttttagtagagacagggtttcaccatgttggccaggctggtctcgaactcctgaccttaggtgatccacctgcctcgacttcccaaagtgctgggattataggcatgagccactgcgcccagtgattatagaaagttaaaggcacatggcaatgcacacgcctatctacgtcttccctgccaaagcaaagggcagcctctgggctcactttcttgcgtttctacttccaaaaggcagtcagaactggcagggccttggagaccacttcatccacctcctagggtccctatgggagagttgaggtccagagcagggaagggtcctgacaggctctgaccagggcctctgatccctacaaacccccaatcggtgtccctctctaccaggacccaagcccacctgctgcagcccactgcctggcc

SEQ ID NO: 5 - DNA, 623 bp, synthetic construct
  misc_feature 1..623: note = Truncated form of the VMD2 promoter
  source 1..623: mol_type = other DNA
aattctgtcattttactagggtgatgaaattcccaagcaacaccatccttttcagataagggcactgaggctgagagaggagctgaaacctacccggcgtcaccacacacaggtggcaaggctgggaccagaaaccaggactgttgactgcagcccggtattcattctttccatagcccacagggctgtcaaagaccccagggcctagtcagaggctcctccttcctggagagttcctggcacagaagttgaagctcagcacagccccctaacccccaactctctctgcaaggcctcaggggtcagaacactggtggagcagatcctttagcctctggattttagggccatggtagagggggtgttgccctaaattccagccctggtctcagcccaacaccctccaagaagaaattagaggggccatggccaggctgtgctagccgttgcttctgagcagattacaagaagggactaagacaaggactcctttgtggaggtcctggcttagggagtcaagtgacggcggctcagcactcacgtgggcagtgccagcctctaagagtgggcaggggcactggccacagagtcccagggagtcccaccagcctagtcgccagacc

SEQ ID NO: 6 - DNA, 462 bp, synthetic construct
  misc_feature 1..462: note = Truncated form of the VMD2 promoter
  source 1..462: mol_type = other DNA
tcattctttccatagcccacagggctgtcaaagaccccagggcctagtcagaggctcctccttcctggagagttcctggcacagaagttgaagctcagcacagccccctaacccccaactctctctgcaaggcctcaggggtcagaacactggtggagcagatcctttagcctctggattttagggccatggtagagggggtgttgccctaaattccagccctggtctcagcccaacaccctccaagaagaaattagaggggccatggccaggctgtgctagccgttgcttctgagcagattacaagaagggactaagacaaggactcctttgtggaggtcctggcttagggagtcaagtgacggcggctcagcactcacgtgggcagtgccagcctctaagagtgggcaggggcactggccacagagtcccagggagtcccaccagcctagtcgccagacc

SEQ ID NO: 7 - DNA, 500 bp, synthetic construct
  misc_feature 1..500: note = Human phosphoglycerate kinase-1 (PGK) promoter
  source 1..500: mol_type = other DNA
gggtaggggaggcgcttttcccaaggcagtctggagcatgcgctttagcagccccgctgggcacttggcgctacacaagtggcctctggcctcgcacacattccacatccaccggtaggcgccaaccggctccgttctttggtggccccttcgcgccaccttctactcctcccctagtcaggaagttcccccccgccccgcagctcgcgtcgtgcaggacgtgacaaatggaagtagcacgtctcactagtctcgtgcagatggacagcaccgctgagcaatggaagcgggtaggcctttggggcagcggccaatagcagctttgctccttcgctttctgggctcagaggctgggaaggggtgggtccgggggcgggctcaggggcgggctcaggggcggggcgggcgcccgaaggtcctccggaggcccggcattctgcacgcttcaaaagcgcacgtctgccgcgctgttctcctcttcctcatctccgggcctttcg

SEQ ID NO: 8 - DNA, 1182 bp, synthetic construct
  misc_feature 1..1182: note = EF1alpha promoter
  source 1..1182: mol_type = other DNA
gctccggtgcccgtcagtgggcagagcgcacatcgcccacagtccccgagaagttggggggaggggtcggcaattgaaccggtgcctagagaaggtggcgcggggtaaactgggaaagtgatgtcgtgtactggctccgcctttttcccgagggtgggggagaaccgtatataagtgcagtagtcgccgtgaacgttctttttcgcaacgggtttgccgccagaacacaggtaagtgccgtgtgtggttcccgcgggcctggcctctttacgggttatggcccttgcgtgccttgaattacttccacgcccctggctgcagtacgtgattcttgatcccgagcttcgggttggaagtgggtgggagagttcgaggccttgcgcttaaggagccccttcgcctcgtgcttgagttgaggcctggcttgggcgctggggccgccgcgtgcgaatctggtggcaccttcgcgcctgtctcgctgctttcgataagtctctagccatttaaaatttttgatgacctgctgcgacgctttttttctggcaagatagtcttgtaaatgcgggccaagatctgcacactggtatttcggtttttggggccgcgggcggcgacggggcccgtgcgtcccagcgcacatgttcggcgaggcggggcctgcgagcgcggccaccgagaatcggacgggggtagtctcaagctggccggcctgctctggtgcctggcctcgcgccgccgtgtatcgccccgccctgggcggcaaggctggcccggtcggcaccagttgcgtgagcggaaagatggccgcttcccggccctgctgcagggagctcaaaatggaggacgcggcgctcgggagagcgggcgggtgagtcacccacacaaaggaaaagggcctttccgtcctcagccgtcgcttcatgtgactccacggagtaccgggcgccgtccaggcacctcgattagttctcgagcttttggagtacgtcgtctttaggttggggggaggggttttatgcgatggagtttccccacactgagtgggtggagactgaagttaggccagcttggcacttgatgtaattctccttggaatttgccctttttgagtttggatcttggttcattctcaagcctcagacagtggttcaaagtttttttcttccatttcaggtgtcgtga

SEQ ID NO: 9 - DNA, 230 bp, synthetic construct
  misc_feature 1..230: note = EF1alpha without the large intron promoter
  source 1..230: mol_type = other DNA
gctccggtgcccgtcagtgggcagagcgcacatcgcccacagtccccgagaagttggggggaggggtcggcaattgaaccggtgcctagagaaggtggcgcggggtaaactgggaaagtgatgtcgtgtactggctccgcctttttcccgagggtgggggagaaccgtatataagtgcagtagtcgccgtgaacgttctttttcgcaacgggtttgccgccagaacacag

SEQ ID NO: 10 - protein, 418 aa, Homo sapiens
MQALVLLLCIGALLGHSSCQNPASPPEEGSPDPDSTGALVEEEDPFFKVPVNKLAAAVSNFGYDLYRVRSSTSPTTNVLLSPLSVATALSALSLGAEQRTESIIHRALYYDLISSPDIHGTYKELLDTVTAPQKNLKSASRIVFEKKLRIKSSFVAPLEKSYGTRPRVLTGNPRLDLQEINNWVQAQMKGKLARSTKEIPDEISILLLGVAHFKGQWVTKFDSRKTSLEDFYLDEERTVRVPMMSDPKAVLRYGLDSDLSCKIAQLPLTGSMSIIFFLPLKVTQNLTLIEESLTSEFIHDIDRELKTVQAVLTVPKLKLSYEGEVTKSLQEMKLQSLFDSPDFSKITGKPIKLTQVEHRAGFEWNEDGAGTTPSPGLQPAHLTFPLDYHLNQPFIFVLRDTDTGALLFIGKILDPRGP

SEQ ID NO: 11 - DNA, 1254 bp, Homo sapiens
  source 1..1254: mol_type = other DNA
atgcaggccctggtgctactcctctgcattggagccctcctcgggcacagcagctgccagaaccctgccagccccccggaggagggctccccagaccccgacagcacaggggcgctggtggaggaggaggatcctttcttcaaagtccccgtgaacaagctggcagcggctgtctccaacttcggctatgacctgtaccgggtgcgatccagcacgagccccacgaccaacgtgctcctgtctcctctcagtgtggccacggccctctcggccctctcgctgggagcggagcagcgaacagaatccatcattcaccgggctctctactatgacttgatcagcagcccagacatccatggtacctataaggagctccttgacacggtcactgccccccagaagaacctcaagagtgcctcccggatcgtctttgagaagaagctgcgcataaaatccagctttgtggcacctctggaaaagtcatatgggaccaggcccagagtcctgacgggcaaccctcgcttggacctgcaagagatcaacaactgggtgcaggcgcagatgaaagggaagctcgccaggtccacaaaggaaattcccgatgagatcagcattctccttctcggtgtggcgcacttcaaggggcagtgggtaacaaagtttgactccagaaagacttccctcgaggatttctacttggatgaagagaggaccgtgagggtccccatgatgtcggaccctaaggctgttttacgctatggcttggattcagatctcagctgcaagattgcccagctgcccttgaccggaagcatgagtatcatcttcttcctgcccctgaaagtgacccagaatttgaccttgatagaggagagcctcacctccgagttcattcatgacatagaccgagaactgaagaccgtgcaggcggtcctcactgtccccaagctgaagctgagttatgaaggcgaagtcaccaagtccctgcaggagatgaagctgcaatccttgtttgattcaccagactttagcaagatcacaggcaaacccatcaagctgactcaggtggaacaccgggctggctttgagtggaacgaggatggggcgggaaccacccccagcccagggctgcagcctgcccacctcaccttcccgctggactatcaccttaaccagcctttcatcttcgtactgagggacacagacacaggggcccttctcttcattggcaagattctggaccccaggggcccc

SEQ ID NO: 12 - DNA, 1254 bp, synthetic construct
  misc_feature 1..1254: note = nucleic acid sequence encoding codon optimised PEDF
  source 1..1254: mol_type = other DNA
atgcaggccctggtgctgctgctgtgcatcggcgccctgctgggccacagcagctgccagaaccccgccagcccccccgaggagggcagccccgaccccgacagcaccggcgccctggtggaggaggaggaccccttcttcaaggtgcccgtgaacaagctggccgccgccgtgagcaacttcggctacgacctgtaccgcgtgcgcagcagcaccagccccaccaccaacgtgctgctgagccccctgagcgtggccaccgccctgagcgccctgagcctgggcgccgagcagcgcaccgagagcatcatccaccgcgccctgtactacgacctgatcagcagccccgacatccacggcacctacaaggagctgctggacaccgtgaccgccccccagaagaacctgaagagcgccagccgcatcgtgttcgagaagaagctgcgcatcaagagcagcttcgtggcccccctggagaagagctacggcacccgcccccgcgtgctgaccggcaacccccgcctggacctgcaggagatcaacaactgggtgcaggcccagatgaagggcaagctggcccgcagcaccaaggagatccccgacgagatcagcatcctgctgctgggcgtggcccacttcaagggccagtgggtgaccaagttcgacagccgcaagaccagcctggaggacttctacctggacgaggagcgcaccgtgcgcgtgcccatgatgagcgaccccaaggccgtgctgcgctacggcctggacagcgacctgagctgcaagatcgcccagctgcccctgaccggcagcatgagcatcatcttcttcctgcccctgaaggtgacccagaacctgaccctgatcgaggagagcctgaccagcgagttcatccacgacatcgaccgcgagctgaagaccgtgcaggccgtgctgaccgtgcccaagctgaagctgagctacgagggcgaggtgaccaagagcctgcaggagatgaagctgcagagcctgttcgacagccccgacttcagcaagatcaccggcaagcccatcaagctgacccaggtggagcaccgcgccggcttcgagtggaacgaggacggcgccggcaccacccccagccccggcctgcagcccgcccacctgaccttccccctggactaccacctgaaccagcccttcatcttcgtgctgcgcgacaccgacaccggcgccctgctgttcatcggcaagatcctggacccccgcggcccc

SEQ ID NO: 13 - DNA, 1254 bp, synthetic construct
  misc_feature 1..1254: note = nucleic acid sequence encoding PEDF comprising a modified signal peptide sequence
  source 1..1254: mol_type = other DNA
atgcgccgcctggtgctgctgctgtgcatcggcgccctgctgggccacgtgttctgccagaaccccgccagcccccccgaggagggcagccccgaccccgacagcaccggcgccctggtggaggaggaggaccccttcttcaaggtgcccgtgaacaagctggccgccgccgtgagcaacttcggctacgacctgtaccgcgtgcgcagcagcaccagccccaccaccaacgtgctgctgagccccctgagcgtggccaccgccctgagcgccctgagcctgggcgccgagcagcgcaccgagagcatcatccaccgcgccctgtactacgacctgatcagcagccccgacatccacggcacctacaaggagctgctggacaccgtgaccgccccccagaagaacctgaagagcgccagccgcatcgtgttcgagaagaagctgcgcatcaagagcagcttcgtggcccccctggagaagagctacggcacccgcccccgcgtgctgaccggcaacccccgcctggacctgcaggagatcaacaactgggtgcaggcccagatgaagggcaagctggcccgcagcaccaaggagatccccgacgagatcagcatcctgctgctgggcgtggcccacttcaagggccagtgggtgaccaagttcgacagccgcaagaccagcctggaggacttctacctggacgaggagcgcaccgtgcgcgtgcccatgatgagcgaccccaaggccgtgctgcgctacggcctggacagcgacctgagctgcaagatcgcccagctgcccctgaccggcagcatgagcatcatcttcttcctgcccctgaaggtgacccagaacctgaccctgatcgaggagagcctgaccagcgagttcatccacgacatcgaccgcgagctgaagaccgtgcaggccgtgctgaccgtgcccaagctgaagctgagctacgagggcgaggtgaccaagagcctgcaggagatgaagctgcagagcctgttcgacagccccgacttcagcaagatcaccggcaagcccatcaagctgacccaggtggagcaccgcgccggcttcgagtggaacgaggacggcgccggcaccacccccagccccggcctgcagcccgcccacctgaccttccccctggactaccacctgaaccagcccttcatcttcgtgctgcgcgacaccgacaccggcgccctgctgttcatcggcaagatcctggacccccgcggcccc

SEQ ID NO: 14 - protein, 242 aa, synthetic construct
  REGION 1..242: note = anti-C3b single chain variable fragment
DIQMTQSPSSLSASVGDRVTITCRASQDVSTAVAWYQQKPGKAPKLLIYSASFLYSGVPSRFSGSGSGTDFTLTISSLQPEDFATYYCQQSYATLPTFEQGTKVEIKRGGGGGSGGGGSGGGGSGGGGSEVQLVESGGGLVQPGGSLRLSCAASGFSFTSSSVSPGKGLEWVGLIYPYNGFNYYADSVKGRFTISADTSLQMNSLRAEDTAVYYCARNALYGSGGYYAMDYWGQGTLVTVSS

SEQ ID NO: 15 - DNA, 726 bp, synthetic construct
  misc_feature 1..726: note = nucleic acid sequence encoding anti-C3b single chain variable fragment
  source 1..726: mol_type = other DNA
gacatccagatgacccagagccccagcagcctgagcgccagcgtgggcgaccgcgtgaccatcacctgccgcgccagccaggacgtaagcaccgccgtggcctggtaccagcagaagcccggcaaggcccccaagctgctgatctacagcgccagcttcctgtacagcggcgtgcccagccgcttcagcggcagcggcagcggcaccgacttcaccctgaccatcagcagcctgcagcccgaggacttcgccacctactactgccagcagagctacgccaccctgcccaccttcgagcagggcaccaaggtggagatcaagcgcggcggcggcggcggcagcggcggcggcggcagcggcggcggcggcagcggcggcggcggcagcgaggtgcagctggtggagagcggcggcggcctggtgcagcccggcggcagcctgcgcctgagctgcgccgccagcggcttcagcttcaccagcagcagcgtgagccccggcaagggcctggagtgggtgggcctgatctacccctacaacggcttcaactactacgccgacagcgtgaagggccgcttcaccatcagcgccgacaccagcctgcagatgaacagcctgcgcgccgaggacaccgccgtgtactactgcgcccgcaacgccctgtacggcagcggcggctactacgccatggactactggggccagggcaccctggtgaccgtgagcagc

SEQ ID NO: 16 - protein, 250 aa, synthetic construct
  REGION 1..250: note = anti-Bb single chain variable fragment
DVQITQSPSYLAASPGETITINCRASKSISKYLAWYQDKPGKTNKLLIYSGSTLQSGIPSRFSGSGSGTDFTLTISSLEPEDFAMYYCQQHDEYPWTFGGGTKLEIKRGGGGGSGGGGSGGGGSGGGGSQVQLQQSGAELAKPGASVRMSCKASGYTFTNYWIHWVKQRPGQGLEWIGYINPNTGYNDYNQKFKDKATLTADKSSSTVYMQLSSLTSEDSAVYYCARGGQLGLRRAMDYWGQGTSVTVSS

SEQ ID NO: 17 - DNA, 750 bp, synthetic construct
  misc_feature 1..750: note = nucleic acid sequence encoding anti-Bb single chain variable fragment
  source 1..750: mol_type = other DNA
gacgtgcagatcacccagagccccagctacctggccgccagccccggcgagaccatcaccatcaactgccgcgccagcaagagcatcagcaagtacctggcctggtaccaggacaagcccggcaagaccaacaagctgctgatctacagcggcagcaccctgcagagcggcatccccagccgcttcagcggcagcggcagcggcaccgacttcaccctgaccatcagcagcctggagcccgaggacttcgccatgtactactgccagcagcacgacgagtacccctggaccttcggcggcggcaccaagctggagatcaagcgcggcggcggcggcggcagcggcggcggcggcagcggcggcggcggcagcggcggcggcggcagccaggtgcagctgcagcagagcggcgccgagctggccaagcccggcgccagcgtgcgcatgagctgcaaggccagcggctacaccttcaccaactactggatccactgggtgaagcagcgccccggccagggcctggagtggatcggctacatcaaccccaacaccggctacaacgactacaaccagaagttcaaggacaaggccaccctgaccgccgacaagagcagcagcaccgtgtacatgcagctgagcagcctgaccagcgaggacagcgccgtgtactactgcgcccgcggcggccagctgggcctgcgccgcgccatggactactggggccagggcaccagcgtgaccgtgagcagc

SEQ ID NO: 18 - protein, 320 aa, synthetic construct
  REGION 1..320: note = soluble form of the normally plasma membrane bound CD55
DCGLPPDVPNAQPALEGRTSFPEDTVITYKCEESFVKIPGEKDSVICLKGSQWSDIEEFCNRSCEVPTRLNSASLKQPYITQNYFPVGTVVEYECRPGYRREPSLSPKLTCLQNLKWSTAVEFCKKKSCPNPGEIRNGQIDVPGGILFGATISFSCNTGYKLFGSTSSFCLISGSSVQWSDPLPECREIYCPAPPQIDNGIIQGERDHYGYRQSVTYACNKGFTMIGEHSIYCTVNNDEGEWSGPPPECRGKSLTSKVPPTVQKPTTVNVPTTEVSPTSQKTTTKTTTPNAQATRSTPVSRTTKHFHETTPNKGSGTTSG

SEQ ID NO: 19 - DNA, 960 bp, synthetic construct
  misc_feature 1..960: note = nucleic acid sequence encoding soluble form of the normally plasma membrane-bound CD55
  source 1..960: mol_type = other DNA
gactgcggcctgccccccgacgtgcccaacgcccagcccgccctggagggccgcaccagcttccccgaggacaccgtgatcacctacaagtgcgaggagagcttcgtgaagatccccggcgagaaggacagcgtgatctgcctgaagggcagccagtggagcgacatcgaggagttctgcaaccgcagctgcgaggtgcccacccgcctgaacagcgccagcctgaagcagccctacatcacccagaactacttccccgtgggcaccgtggtggagtacgagtgccgccccggctaccgccgcgagcccagcctgagccccaagctgacctgcctgcagaacctgaagtggagcaccgccgtggagttctgcaagaagaagagctgccccaaccccggcgagatccgcaacggccagatcgacgtgcccggcggcatcctgttcggcgccaccatcagcttcagctgcaacaccggctacaagctgttcggcagcaccagcagcttctgcctgatcagcggcagcagcgtgcagtggagcgaccccctgcccgagtgccgcgagatctactgccccgcccccccccagatcgacaacggcatcatccagggcgagcgcgaccactacggctaccgccagagcgtgacctacgcctgcaacaagggcttcaccatgatcggcgagcacagcatctactgcaccgtgaacaacgacgagggcgagtggagcggccccccccccgagtgccgaggcaagagcctgaccagcaaggtgccccccaccgtgcagaagcccaccaccgtgaacgtgcccaccaccgaggtgagccccaccagccagaagaccaccaccaagaccaccacccccaacgcccaggccacccgcagcacccccgtgagccgcaccaccaagcacttccacgagaccacccccaacaagggcagcggcaccaccagcggc

SEQ ID NO: 20 - protein, 312 aa, Homo sapiens
EATFCDFPKINHGILYDEEKYKPFSQVPTGEVFYYSCEYNFVSPSKSFWTRITCTEEGWSPTPKCLRLCFFPFVENGHSESSGQTHLEGDTVQIICNTGYRLQNNENNISCVERGWSTPPKCRSTDTSCVNPPTVQNAHILSRQMSKYPSGERVRYECRSPYEMFGDEEVMCLNGNWTEPPQCKDSTGKCGPPPPIDNGDITSFPLSVYAPASSVEYQCQNLYQLEGNKRITCRNGQWSEPPKCLHPCVISREIMENYNIALRWTAKQKLYLRTGESAEFVCKRGYRLSSRSHTLRTTCWDGKLEYPTCAKR

SEQ ID NO: 21 - DNA, 936 bp, Homo sapiens
  source 1..936: mol_type = other DNA
gaagcaacattttgtgattttccaaaaataaaccatggaattctatatgatgaagaaaaatataagccattttcccaggttcctacaggggaagttttctattactcctgtgaatataattttgtgtctccttcaaaatcattttggactcgcataacatgcacagaagaaggatggtcaccaacaccaaagtgtctcagactgtgtttctttccttttgtggaaaatggtcattctgaatcttcaggacaaacacatctggaaggtgatactgtgcaaattatttgcaacacaggatacagacttcaaaacaatgagaacaacatttcatgtgtagaacggggctggtccacccctcccaaatgcaggtccactgacacttcctgtgtgaatccgcccacagtacaaaatgctcatatactgtcgagacagatgagtaaatatccatctggtgagagagtacgttatgaatgtaggagcccttatgaaatgtttggggatgaagaagtgatgtgtttaaatggaaactggacagaaccacctcaatgcaaagattctacgggaaaatgtgggccccctccacctattgacaatggggacattacttcattcccgttgtcagtatatgctccagcttcatcagttgagtaccaatgccagaacttgtatcaacttgagggtaacaagcgaataacatgtagaaatggacaatggtcagaaccaccaaaatgcttacatccgtgtgtaatatcccgagaaattatggaaaattataacatagcattaaggtggacagccaaacagaagctttatttgagaacaggtgaatcagctgaatttgtgtgtaaacggggatatcgtctttcatcacgttctcacacattgcgaacaacatgttgggatgggaaactggagtatccaacttgtgcaaaaaga

SEQ ID NO: 22 - DNA, 936 bp, synthetic construct
  misc_feature 1..936: note = codon optimised nucleic acid sequence encoding human complement factor H related protein-1 (CFHR1)
  source 1..936: mol_type = other DNA
gaggccaccttctgcgacttccccaagatcaaccacggcatcctgtacgacgaggagaagtacaagcccttcagccaggtgcccaccggcgaggtgttctactacagctgcgagtacaacttcgtgagccccagcaagagcttctggacccgcatcacctgcaccgaggagggctggagccccacccccaagtgcctgcgcctgtgcttcttccccttcgtggagaacggccacagcgagagcagcggccagacccacctggagggcgacaccgtgcagatcatctgcaacaccggctaccgcctgcagaacaacgagaacaacatcagctgcgtggagcgcggctggagcaccccccccaagtgccgcagcaccgacaccagctgcgtgaacccccccaccgtgcagaacgcccacatcctgagccgccagatgagcaagtaccccagcggcgagcgcgtgcgctacgagtgccgcagcccctacgagatgttcggcgacgaggaggtgatgtgcctgaacggcaactggaccgagcccccccagtgcaaggacagcaccggcaagtgcggcccccccccccccatcgacaacggcgacatcaccagcttccccctgagcgtgtacgcccccgccagcagcgtggagtaccagtgccagaacctgtaccagctggagggcaacaagcgcatcacctgccgcaacggccagtggagcgagccccccaagtgcctgcacccctgcgtgatcagccgcgagatcatggagaactacaacatcgccctgcgctggaccgccaagcagaagctgtacctgcgcaccggcgagagcgccgagttcgtgtgcaagcgcggctaccgcctgagcagccgcagccacaccctgcgcaccacctgctgggacggcaagctggagtaccccacctgcgccaagcgc

SEQ ID NO: 23 - protein, 310 aa, synthetic construct
  REGION 1..310: note = soluble form of the normally plasma membrane-bound CD46 (sCD46)
CEEPPTFEAMELIGKPKPYYEIGERVDYKCKKGYFYIPPLATHTICDRNHTWLPVSDDACYRETCPYIRDPLNGQAVPANGTYEFGYQMHFICNEGYYLIGEEILYCELKGSVAIWSGKPPICEKVLCTPPPKIKNGKHTFSEVEVFEYLDAVTYSCDPAPGPDPFSLIGESTIYCGDNSVWSRAAPECKVVKCRFPVVENGKQISGFGKKFYYKATVMFECDKGFYLDGSDTIVCDSNSTWDPPVPKCLKVLPPSSTKPPALSHSVSTSSTTKSPASSASGPRPTYKPPVSNYPGYPKPEEGILDSLDV

SEQ ID NO: 24 - DNA, 930 bp, synthetic construct
  misc_feature 1..930: note = nucleic acid sequence encoding a soluble form of the normally plasma membrane-bound CD46 (sCD46)
  source 1..930: mol_type = other DNA
tgcgaggagccccccaccttcgaggccatggagctgatcggcaagcccaagccctactacgagatcggcgagcgcgtggactacaagtgcaagaagggctacttctacatcccccccctggccacccacaccatctgcgaccgcaaccacacctggctgcccgtgagcgacgacgcctgctaccgcgagacctgcccctacatccgcgaccccctgaacggccaggccgtgcccgccaacggcacctacgagttcggctaccagatgcacttcatctgcaacgagggctactacctgatcggcgaggagatcctgtactgcgagctgaagggcagcgtggccatctggagcggcaagccccccatctgcgagaaggtgctgtgcacccccccccccaagatcaagaacggcaagcacaccttcagcgaggtggaggtgttcgagtacctggacgccgtgacctacagctgcgaccccgcccccggccccgaccccttcagcctgatcggcgagagcaccatctactgcggcgacaacagcgtgtggagccgcgccgcccccgagtgcaaggtggtgaagtgccgcttccccgtggtggagaacggcaagcagatcagcggcttcggcaagaagttctactacaaggccaccgtgatgttcgagtgcgacaagggcttctacctggacggcagcgacaccatcgtgtgcgacagcaacagcacctgggacccccccgtgcccaagtgcctgaaggtgctgccccccagcagcaccaagccccccgccctgagccacagcgtgagcaccagcagcaccaccaagagccccgccagcagcgccagcggcccccgccccacctacaagccccccgtgagcaactaccccggctaccccaagcccgaggagggcatcctggacagcctggacgtg

SEQ ID NO: 25 - protein, 19 aa, synthetic construct
  REGION 1..19: note = P2A peptide spacer sequence
ATNFSLLKQAGDVEENPGP

SEQ ID NO: 26 - DNA, 57 bp, synthetic construct
  misc_feature 1..57: note = nucleic acid sequence encoding P2A peptide spacer sequence
  source 1..57: mol_type = other DNA
gccaccaacttcagcctgctgaagcaggccggcgacgtggaggagaaccccggcccc

SEQ ID NO: 27 - protein, 20 aa, synthetic construct
  REGION 1..20: note = E2A peptide spacer sequence
QCTNYALLKLAGDVESNPGP

SEQ ID NO: 28 - DNA, 60 bp, synthetic construct
  misc_feature 1..60: note = nucleic acid sequence encoding E2A peptide spacer sequence
  source 1..60: mol_type = other DNA
cagtgcaccaactacgccctgctgaagctggccggcgacgtggagagcaaccccggcccc

SEQ ID NO: 29 - protein, 18 aa, synthetic construct
  REGION 1..18: note = T2A peptide spacer sequence
EGRGSLLTCGDVEENPGP

SEQ ID NO: 30 - DNA, 54 bp, synthetic construct
  misc_feature 1..54: note = nucleic acid sequence encoding T2A peptide spacer sequence
  source 1..54: mol_type = other DNA
gagggccgcggcagcctgctgacctgcggcgacgtggaggagaaccccggcccc

SEQ ID NO: 31 - protein, 22 aa, synthetic construct
  REGION 1..22: note = F2A peptide spacer sequence
VKQTLNFDLLKLAGDVESNPGP

SEQ ID NO: 32 - DNA, 66 bp, synthetic construct
  misc_feature 1..66: note = nucliec acid sequence encoding F2A peptide spacer sequence
  source 1..66: mol_type = other DNA
gtgaagcagaccctgaacttcgacctgctgaagctggccggcgacgtggagagcaaccccggcccc

SEQ ID NO: 33 - skipped

SEQ ID NO: 34 - protein, 9 aa, synthetic construct
  REGION 1..9: note = viral-2A removal sequence wherein the hydrophilic amino acid is serine
RRSKRSGSG

SEQ ID NO: 35 - DNA, 27 bp, synthetic construct
  misc_feature 1..27: note = nucleic acid sequence encoding viral-2A removal sequence wherein the hydrophilic amino acid is serine
  source 1..27: mol_type = other DNA
cgccgcagcaagcgcagcggcagcggc

SEQ ID NO: 36 - protein, 9 aa, synthetic construct
  REGION 1..9: note = viral-2A removal sequence wherein the hydrophilic amino acid is threonine
RRTKRSGSG

SEQ ID NO: 37 - DNA, 27 bp, synthetic construct
  misc_feature 1..27: note = nucleic acid sequence encoding viral-2A removal sequence wherein the hydrophilic amino acid is threonine
  source 1..27: mol_type = other DNA
cgccgcaccaagcgcagcggcagcggc

SEQ ID NO: 38 - protein, 11 aa, synthetic construct
  REGION 1..11: note = viral-2A removal sequence which comprises a gelatinase MMP-2 recognition sequence and the tripeptide GSG linker sequence
GPQGIAGQGSG

SEQ ID NO: 39 - DNA, 33 bp, synthetic construct
  misc_feature 1..33: note = nucleic acid sequence encoding viral-2A removal sequence which comprises a gelatinase MMP-2 recognition sequence and the tripeptide GSG linker sequence
  source 1..33: mol_type = other DNA
ggccccctgggcatcgccggccagggcagcggc

SEQ ID NO: 40 - protein, 12 aa, synthetic construct
  REGION 1..12: note = viral-2A removal sequence which comprises a renin recognition sequence and the tripeptide GSG linker sequence
HPFHLLVYSGSG

SEQ ID NO: 41 - DNA, 36 bp, synthetic construct
  misc_feature 1..36: note = nucleic acid sequence encoding viral-2A removal sequence which comprises a renin recognition sequence and the tripeptide GSG linker sequence
  source 1..36: mol_type = other DNA
cgccccttccacctgctggtcatccacggcagcggc

SEQ ID NO: 42 - DNA, 592 bp, synthetic construct
  misc_feature 1..592: note = Woodchuck Hepatitis Virus Post-transcriptional Regulatory Element (WPRE)
  source 1..592: mol_type = other DNA
aatcaacctctggattacaaaatttgtgaaagattgactggtattcttaactatgttgctccttttacgctatgtggatacgctgctttaatgcctttgtatcatgctattgcttcccgtatggctttcattttctcctccttgtataaatcctggttgctgtctctttatgaggagttgtggcccgttgtcaggcaacgtggcgtggtgtgcactgtgtttgctgacgcaacccccactggttggggcattgccaccacctgtcagctcctttccgggactttcgctttccccctccctattgccacggcggaactcatcgccgcctgccttgcccgctgctggacaggggctcggctgttgggcactgacaattccgtggtgttgtcggggaagctgacgtcctttccatggctgctcgcctgtgttgccacctggattctgcgcgggacgtccttctgctacgtcccttcggccctcaatccagcggaccttccttcccgcggcctgctgccggctctgcggcctcttccgcgtcttcgccttcgccctcagacgagtcggatctccctttgggccgcctccccgcctg

SEQ ID NO: 43 - DNA, 247 bp, synthetic construct
  misc_feature 1..247: note = truncated WPRE
  source 1..247: mol_type = other DNA
aatcaacctctggattacaaaatttgtgaaagattgactggtattcttaactatgttgctccttttacgctatgtggatacgctgctttaatgcctttgtatcatgctattgcttcccgtatggctttcattttctcctccttgtataaatcctggttagttcttgccacggcggaactcatcgccgcctgccttgcccgctgctggacaggggctcggctgttgggcactgacaattccgtggtgt

SEQ ID NO: 44 - DNA, 224 bp, synthetic construct
  misc_feature 1..224: note = simian virus-40 poly-A nucleotide sequence
  source 1..224: mol_type = other DNA
agcagacatgataagatacattgatgagtttggacaaaccacaactagaatgcagtgaaaaaaatgctttatttgtgaaatttgtgatgctattgctttatttgtaaccattataagctgcaataaacaagttaacaacaacaattgcattcattttatgtttcaggttcagggggaggtgtgggaggttttttaaagcaagtaaaacctctacaaatgtggta

SEQ ID NO: 45 - DNA, 169 bp, synthetic construct
  misc_feature 1..169: note = poly-A component
  source 1..169: mol_type = other DNA
ttcgagcaacttgtttattgcagcttataatggttacaaataaagcaatagcatcacaaatttcacaaataaagcatttttttcactgcattctagttgtggtttgtccaaactcatcaatgtatcttatcatgtctggatcgtctagcatcgaagatcccccgatctg

SEQ ID NO: 46 - DNA, 129 bp, synthetic construct
  misc_feature 1..129: note = left Inverted Terminal Repeat (ITR) sequence taken from a commercially available recombinant AAV genome plasmid
  source 1..129: mol_type = other DNA
cgcgctcgctcgctcactgaggccgcccgggcaaagcccgggcgtcgggcgacctttggtcgcccggcctcagtgagcgagcgagcgcgcagagagggagtggccaactccatcactaggggttccttg

SEQ ID NO: 47 - DNA, 128 bp, synthetic construct
  misc_feature 1..128: note = right Inverted Terminal Repeat (ITR) sequence taken from a commercially available recombinant AAV genome plasmid
  source 1..128: mol_type = other DNA
aggaacccctagtgatggagttggccactccctctctgcgcgctcgctcgctcactgaggccgggcgaccaaaggtcgcccgacgcccgggctttgcccgggcggcctcagtgagcgagcgagcgcgc

SEQ ID NO: 48 - DNA, 121 bp, synthetic construct
  misc_feature 1..121: note = minute virus of mice (MVM) small intron
  source 1..121: mol_type = other DNA
aggtacgatggcgcctccagctaaaagagctaaaagaggtaagggtttaagggatggttggttggtggggtattaatgtttaattacctgttttacaggcctgaaatcacttggttttagg

SEQ ID NO: 49 - DNA, 133 bp, synthetic construct
  misc_feature 1..133: note = nucliec acid sequence from the 5'-donor sites of the first intron of the human beta-globin gene and the branch and 3'-acceptor sites from the intron of an immunoglobulin gene heavy chain variable region
  source 1..133: mol_type = other DNA
gtaagtatcaaggttacaagacaggtttaaggagaccaatagaaactgggcttgtcgagacagagaagactcttgcgtttctgataggcacctattggtcttactgacatccactttgcctttctctccacag

SEQ ID NO: 50 - DNA, 210 bp, synthetic construct
  misc_feature 1..210: note = a fusion of 5' and 3' nucleotide components of the splice acceptor of the rabbit beta-globulin gene 1
  source 1..210: mol_type = other DNA
gtgagcgggcgggacggcccttctcctccgggctgtaattagcgcttggtttaatgacggcttgtttcttttctgtggctgcgtgaaagccttgaggggctccgggaggctagagcctctgctaaccatgttcatgccttcttctttttcctacagctcctgggcaacgtgctggttattgtgctgtctcatcattttggcaaagaattc

SEQ ID NO: 51 - protein, 19 aa, synthetic construct
  REGION 1..19: note = signal peptide
MRRLVLLLCIGALLGHVFC

SEQ ID NO: 52 - DNA, 57 bp, synthetic construct
  misc_feature 1..57: note = nucleic acid encoding signal peptide of SEQ ID NO: 51
  source 1..57: mol_type = other DNA
atgcgccgcctggtgctgctgctgtgcatcggcgccctgctgggccacgtgttctgc

SEQ ID NO: 53 - protein, 19 aa, synthetic construct
  REGION 1..19: note = signal peptide
MRRFLTVISFLLYFGCAFA

SEQ ID NO: 54 - DNA, 57 bp, synthetic construct
  misc_feature 1..57: note = nucleic acid encoding signal peptide of SEQ ID NO: 53
  source 1..57: mol_type = other DNA
atgcgccgcttcctgaccgtgatcagcttcctgctgtacttcggctgcgccttcgcc

SEQ ID NO: 55 - protein, 706 aa, synthetic construct
  REGION 1..706: note = PEDF-furin-P2A-anti-C3b SCVF
MRRLVLLLCIGALLGHVFCQNPASPPEEGSPDPDSTGALVEEEDPFFKVPVNKLAAAVSNFGYDLYRVRSSTSPTTNVLLSPLSVATALSALSLGAEQRTESIIHRALYYDLISSPDIHGTYKELLDTVTAPQKNLKSASRIVFEKKLRIKSSFVAPLEKSYGTRPRVLTGNPRLDLQEINNWVQAQMKGKLARSTKEIPDEISILLLGVAHFKGQWVTKFDSRKTSLEDFYLDEERTVRVPMMSDPKAVLRYGLDSDLSCKIAQLPLTGSMSIIFFLPLKVTQNLTLIEESLTSEFIHDIDRELKTVQAVLTVPKLKLSYEGEVTKSLQEMKLQSLFDSPDFSKITGKPIKLTQVEHRAGFEWNEDGAGTTPSPGLQPAHLTFPLDYHLNQPFIFVLRDTDTGALLFIGKILDPRGPRRSKRSGSGATNFSLLKQAGDVEENPGPMRRLLTFISILALVGAFADIQMTQSPSSLSASVGDRVTITCRASQDVSTAVAWYQQKPGKAPKLLIYSASFLYSGVPSRFSGSGSGTDFTLTISSLQPEDFATYYCQQSYATLPTFEQGTKVEIKRGGGGGSGGGGSGGGGSGGGGSEVQLVESGGGLVQPGGSLRLSCAASGFSFTSSSVSPGKGLEWVGLIYPYNGFNYYADSVKGRFTISADTSLQMNSLRAEDTAVYYCARNALYGSGGYYAMDYWGQGTLVTVSS

SEQ ID NO: 56 - DNA, 2121 bp, synthetic construct
  misc_feature 1..2121: note = nucleic acid encoding PEDF-furin-P2A-anti-C3b SCVF
  source 1..2121: mol_type = other DNA
atgcgccgcctggtgctgctgctgtgcatcggcgccctgctgggccacgtgttctgccagaaccccgccagcccccccgaggagggcagccccgaccccgacagcaccggcgccctggtggaggaggaggaccccttcttcaaggtgcccgtgaacaagctggccgccgccgtgagcaacttcggctacgacctgtaccgcgtgcgcagcagcaccagccccaccaccaacgtgctgctgagccccctgagcgtggccaccgccctgagcgccctgagcctgggcgccgagcagcgcaccgagagcatcatccaccgcgccctgtactacgacctgatcagcagccccgacatccacggcacctacaaggagctgctggacaccgtgaccgccccccagaagaacctgaagagcgccagccgcatcgtgttcgagaagaagctgcgcatcaagagcagcttcgtggcccccctggagaagagctacggcacccgcccccgcgtgctgaccggcaacccccgcctggacctgcaggagatcaacaactgggtgcaggcccagatgaagggcaagctggcccgcagcaccaaggagatccccgacgagatcagcatcctgctgctgggcgtggcccacttcaagggccagtgggtgaccaagttcgacagccgcaagaccagcctggaggacttctacctggacgaggagcgcaccgtgcgcgtgcccatgatgagcgaccccaaggccgtgctgcgctacggcctggacagcgacctgagctgcaagatcgcccagctgcccctgaccggcagcatgagcatcatcttcttcctgcccctgaaggtgacccagaacctgaccctgatcgaggagagcctgaccagcgagttcatccacgacatcgaccgcgagctgaagaccgtgcaggccgtgctgaccgtgcccaagctgaagctgagctacgagggcgaggtgaccaagagcctgcaggagatgaagctgcagagcctgttcgacagccccgacttcagcaagatcaccggcaagcccatcaagctgacccaggtggagcaccgcgccggcttcgagtggaacgaggacggcgccggcaccacccccagccccggcctgcagcccgcccacctgaccttccccctggactaccacctgaaccagcccttcatcttcgtgctgcgcgacaccgacaccggcgccctgctgttcatcggcaagatcctggacccccgcggcccccgccgcagcaagcgcagcggcagcggcgccaccaacttcagcctgctgaagcaggccggcgacgtggaggagaaccccggccccatgcgccgcctgctgaccttcatcagcatcctggccctggtgggcgccttcgccgacatccagatgacccagagccccagcagcctgagcgccagcgtgggcgaccgcgtgaccatcacctgccgcgccagccaggacgtaagcaccgccgtggcctggtaccagcagaagcccggcaaggcccccaagctgctgatctacagcgccagcttcctgtacagcggcgtgcccagccgcttcagcggcagcggcagcggcaccgacttcaccctgaccatcagcagcctgcagcccgaggacttcgccacctactactgccagcagagctacgccaccctgcccaccttcgagcagggcaccaaggtggagatcaagcgcggcggcggcggcggcagcggcggcggcggcagcggcggcggcggcagcggcggcggcggcagcgaggtgcagctggtggagagcggcggcggcctggtgcagcccggcggcagcctgcgcctgagctgcgccgccagcggcttcagcttcaccagcagcagcgtgagccccggcaagggcctggagtgggtgggcctgatctacccctacaacggcttcaactactacgccgacagcgtgaagggccgcttcaccatcagcgccgacaccagcctgcagatgaacagcctgcgcgccgaggacaccgccgtgtactactgcgcccgcaacgccctgtacggcagcggcggctactacgccatggactactggggccagggcaccctggtgaccgtgagcagctga

SEQ ID NO: 57 - protein, 785 aa, synthetic construct
  REGION 1..785: note = PEDF-furin-P2A-sCD55
MRRLVLLLCIGALLGHVFCQNPASPPEEGSPDPDSTGALVEEEDPFFKVPVNKLAAAVSNFGYDLYRVRSSTSPTTNVLLSPLSVATALSALSLGAEQRTESIIHRALYYDLISSPDIHGTYKELLDTVTAPQKNLKSASRIVFEKKLRIKSSFVAPLEKSYGTRPRVLTGNPRLDLQEINNWVQAQMKGKLARSTKEIPDEISILLLGVAHFKGQWVTKFDSRKTSLEDFYLDEERTVRVPMMSDPKAVLRYGLDSDLSCKIAQLPLTGSMSIIFFLPLKVTQNLTLIEESLTSEFIHDIDRELKTVQAVLTVPKLKLSYEGEVTKSLQEMKLQSLFDSPDFSKITGKPIKLTQVEHRAGFEWNEDGAGTTPSPGLQPAHLTFPLDYHLNQPFIFVLRDTDTGALLFIGKILDPRGPRRSKRSGSGATNFSLLKQAGDVEENPGPMRRFLTVISFLLYFGCAFADCGLPPDVPNAQPALEGRTSFPEDTVITYKCEESFVKIPGEKDSVICLKGSQWSDIEEFCNRSCEVPTRLNSASLKQPYITQNYFPVGTVVEYECRPGYRREPSLSPKLTCLQNLKWSTAVEFCKKKSCPNPGEIRNGQIDVPGGILFGATISFSCNTGYKLFGSTSSFCLISGSSVQWSDPLPECREIYCPAPPQIDNGIIQGERDHYGYRQSVTYACNKGFTMIGEHSIYCTVNNDEGEWSGPPPECRGKSLTSKVPPTVQKPTTVNVPTTEVSPTSQKTTTKTTTPNAQATRSTPVSRTTKHFHETTPNKGSGTTSG

SEQ ID NO: 58 - DNA, 2358 bp, synthetic construct
  misc_feature 1..2358: note = nucleic acid encoding PEDF-furin-P2A-sCD55
  source 1..2358: mol_type = other DNA
atgcgccgcctggtgctgctgctgtgcatcggcgccctgctgggccacgtgttctgccagaaccccgccagcccccccgaggagggcagccccgaccccgacagcaccggcgccctggtggaggaggaggaccccttcttcaaggtgcccgtgaacaagctggccgccgccgtgagcaacttcggctacgacctgtaccgcgtgcgcagcagcaccagccccaccaccaacgtgctgctgagccccctgagcgtggccaccgccctgagcgccctgagcctgggcgccgagcagcgcaccgagagcatcatccaccgcgccctgtactacgacctgatcagcagccccgacatccacggcacctacaaggagctgctggacaccgtgaccgccccccagaagaacctgaagagcgccagccgcatcgtgttcgagaagaagctgcgcatcaagagcagcttcgtggcccccctggagaagagctacggcacccgcccccgcgtgctgaccggcaacccccgcctggacctgcaggagatcaacaactgggtgcaggcccagatgaagggcaagctggcccgcagcaccaaggagatccccgacgagatcagcatcctgctgctgggcgtggcccacttcaagggccagtgggtgaccaagttcgacagccgcaagaccagcctggaggacttctacctggacgaggagcgcaccgtgcgcgtgcccatgatgagcgaccccaaggccgtgctgcgctacggcctggacagcgacctgagctgcaagatcgcccagctgcccctgaccggcagcatgagcatcatcttcttcctgcccctgaaggtgacccagaacctgaccctgatcgaggagagcctgaccagcgagttcatccacgacatcgaccgcgagctgaagaccgtgcaggccgtgctgaccgtgcccaagctgaagctgagctacgagggcgaggtgaccaagagcctgcaggagatgaagctgcagagcctgttcgacagccccgacttcagcaagatcaccggcaagcccatcaagctgacccaggtggagcaccgcgccggcttcgagtggaacgaggacggcgccggcaccacccccagccccggcctgcagcccgcccacctgaccttccccctggactaccacctgaaccagcccttcatcttcgtgctgcgcgacaccgacaccggcgccctgctgttcatcggcaagatcctggacccccgcggcccccgccgcagcaagcgcagcggcagcggcgccaccaacttcagcctgctgaagcaggccggcgacgtggaggagaaccccggccccatgcgccgcttcctgaccgtgatcagcttcctgctgtacttcggctgcgccttcgccgactgcggcctgccccccgacgtgcccaacgcccagcccgccctggagggccgcaccagcttccccgaggacaccgtgatcacctacaagtgcgaggagagcttcgtgaagatccccggcgagaaggacagcgtgatctgcctgaagggcagccagtggagcgacatcgaggagttctgcaaccgcagctgcgaggtgcccacccgcctgaacagcgccagcctgaagcagccctacatcacccagaactacttccccgtgggcaccgtggtggagtacgagtgccgccccggctaccgccgcgagcccagcctgagccccaagctgacctgcctgcagaacctgaagtggagcaccgccgtggagttctgcaagaagaagagctgccccaaccccggcgagatccgcaacggccagatcgacgtgcccggcggcatcctgttcggcgccaccatcagcttcagctgcaacaccggctacaagctgttcggcagcaccagcagcttctgcctgatcagcggcagcagcgtgcagtggagcgaccccctgcccgagtgccgcgagatctactgccccgcccccccccagatcgacaacggcatcatccagggcgagcgcgaccactacggctaccgccagagcgtgacctacgcctgcaacaagggcttcaccatgatcggcgagcacagcatctactgcaccgtgaacaacgacgagggcgagtggagcggccccccccccgagtgccgaggcaagagcctgaccagcaaggtgccccccaccgtgcagaagcccaccaccgtgaacgtgcccaccaccgaggtgagccccaccagccagaagaccaccaccaagaccaccacccccaacgcccaggccacccgcagcacccccgtgagccgcaccaccaagcacttccacgagaccacccccaacaagggcagcggcaccaccagcggctaa

SEQ ID NO: 59 - protein, 785 aa, synthetic construct
  REGION 1..785: note = sCD55-furin-P2A-PEDF
MRRFLTVISFLLYFGCAFADCGLPPDVPNAQPALEGRTSFPEDTVITYKCEESFVKIPGEKDSVICLKGSQWSDIEEFCNRSCEVPTRLNSASLKQPYITQNYFPVGTVVEYECRPGYRREPSLSPKLTCLQNLKWSTAVEFCKKKSCPNPGEIRNGQIDVPGGILFGATISFSCNTGYKLFGSTSSFCLISGSSVQWSDPLPECREIYCPAPPQIDNGIIQGERDHYGYRQSVTYACNKGFTMIGEHSIYCTVNNDEGEWSGPPPECRGKSLTSKVPPTVQKPTTVNVPTTEVSPTSQKTTTKTTTPNAQATRSTPVSRTTKHFHETTPNKGSGTTSGRRSKRSGSGATNFSLLKQAGDVEENPGPMRRLVLLLCIGALLGHVFCQNPASPPEEGSPDPDSTGALVEEEDPFFKVPVNKLAAAVSNFGYDLYRVRSSTSPTTNVLLSPLSVATALSALSLGAEQRTESIIHRALYYDLISSPDIHGTYKELLDTVTAPQKNLKSASRIVFEKKLRIKSSFVAPLEKSYGTRPRVLTGNPRLDLQEINNWVQAQMKGKLARSTKEIPDEISILLLGVAHFKGQWVTKFDSRKTSLEDFYLDEERTVRVPMMSDPKAVLRYGLDSDLSCKIAQLPLTGSMSIIFFLPLKVTQNLTLIEESLTSEFIHDIDRELKTVQAVLTVPKLKLSYEGEVTKSLQEMKLQSLFDSPDFSKITGKPIKLTQVEHRAGFEWNEDGAGTTPSPGLQPAHLTFPLDYHLNQPFIFVLRDTDTGALLFIGKILDPRGP

SEQ ID NO: 60 - DNA, 2358 bp, synthetic construct
  misc_feature 1..2358: note = nucleic acid sequence encoding sCD55-furin-P2A-PEDF
  source 1..2358: mol_type = other DNA
atgcgccgcttcctgaccgtgatcagcttcctgctgtacttcggctgcgccttcgccgactgcggcctgccccccgacgtgcccaacgcccagcccgccctggagggccgcaccagcttccccgaggacaccgtgatcacctacaagtgcgaggagagcttcgtgaagatccccggcgagaaggacagcgtgatctgcctgaagggcagccagtggagcgacatcgaggagttctgcaaccgcagctgcgaggtgcccacccgcctgaacagcgccagcctgaagcagccctacatcacccagaactacttccccgtgggcaccgtggtggagtacgagtgccgccccggctaccgccgcgagcccagcctgagccccaagctgacctgcctgcagaacctgaagtggagcaccgccgtggagttctgcaagaagaagagctgccccaaccccggcgagatccgcaacggccagatcgacgtgcccggcggcatcctgttcggcgccaccatcagcttcagctgcaacaccggctacaagctgttcggcagcaccagcagcttctgcctgatcagcggcagcagcgtgcagtggagcgaccccctgcccgagtgccgcgagatctactgccccgcccccccccagatcgacaacggcatcatccagggcgagcgcgaccactacggctaccgccagagcgtgacctacgcctgcaacaagggcttcaccatgatcggcgagcacagcatctactgcaccgtgaacaacgacgagggcgagtggagcggccccccccccgagtgccgaggcaagagcctgaccagcaaggtgccccccaccgtgcagaagcccaccaccgtgaacgtgcccaccaccgaggtgagccccaccagccagaagaccaccaccaagaccaccacccccaacgcccaggccacccgcagcacccccgtgagccgcaccaccaagcacttccacgagaccacccccaacaagggcagcggcaccaccagcggccgccgcagcaagcgcagcggcagcggcgccaccaacttcagcctgctgaagcaggccggcgacgtggaggagaaccccggccccatgcgccgcctggtgctgctgctgtgcatcggcgccctgctgggccacgtgttctgccagaaccccgccagcccccccgaggagggcagccccgaccccgacagcaccggcgccctggtggaggaggaggaccccttcttcaaggtgcccgtgaacaagctggccgccgccgtgagcaacttcggctacgacctgtaccgcgtgcgcagcagcaccagccccaccaccaacgtgctgctgagccccctgagcgtggccaccgccctgagcgccctgagcctgggcgccgagcagcgcaccgagagcatcatccaccgcgccctgtactacgacctgatcagcagccccgacatccacggcacctacaaggagctgctggacaccgtgaccgccccccagaagaacctgaagagcgccagccgcatcgtgttcgagaagaagctgcgcatcaagagcagcttcgtggcccccctggagaagagctacggcacccgcccccgcgtgctgaccggcaacccccgcctggacctgcaggagatcaacaactgggtgcaggcccagatgaagggcaagctggcccgcagcaccaaggagatccccgacgagatcagcatcctgctgctgggcgtggcccacttcaagggccagtgggtgaccaagttcgacagccgcaagaccagcctggaggacttctacctggacgaggagcgcaccgtgcgcgtgcccatgatgagcgaccccaaggccgtgctgcgctacggcctggacagcgacctgagctgcaagatcgcccagctgcccctgaccggcagcatgagcatcatcttcttcctgcccctgaaggtgacccagaacctgaccctgatcgaggagagcctgaccagcgagttcatccacgacatcgaccgcgagctgaagaccgtgcaggccgtgctgaccgtgcccaagctgaagctgagctacgagggcgaggtgaccaagagcctgcaggagatgaagctgcagagcctgttcgacagccccgacttcagcaagatcaccggcaagcccatcaagctgacccaggtggagcaccgcgccggcttcgagtggaacgaggacggcgccggcaccacccccagccccggcctgcagcccgcccacctgaccttccccctggactaccacctgaaccagcccttcatcttcgtgctgcgcgacaccgacaccggcgccctgctgttcatcggcaagatcctggacccccgcggcccctaa

SEQ ID NO: 61 - protein, 777 aa, synthetic construct
  REGION 1..777: note = PEDF-furin-P2A-CFHR1
MRRLVLLLCIGALLGHVFCQNPASPPEEGSPDPDSTGALVEEEDPFFKVPVNKLAAAVSNFGYDLYRVRSSTSPTTNVLLSPLSVATALSALSLGAEQRTESIIHRALYYDLISSPDIHGTYKELLDTVTAPQKNLKSASRIVFEKKLRIKSSFVAPLEKSYGTRPRVLTGNPRLDLQEINNWVQAQMKGKLARSTKEIPDEISILLLGVAHFKGQWVTKFDSRKTSLEDFYLDEERTVRVPMMSDPKAVLRYGLDSDLSCKIAQLPLTGSMSIIFFLPLKVTQNLTLIEESLTSEFIHDIDRELKTVQAVLTVPKLKLSYEGEVTKSLQEMKLQSLFDSPDFSKITGKPIKLTQVEHRAGFEWNEDGAGTTPSPGLQPAHLTFPLDYHLNQPFIFVLRDTDTGALLFIGKILDPRGPRRSKRSGSGATNFSLLKQAGDVEENPGPMRRFLTVISFLLYFGCAFAEATFCDFPKINHGILYDEEKYKPFSQVPTGEVFYYSCEYNFVSPSKSFWTRITCTEEGWSPTPKCLRLCFFPFVENGHSESSGQTHLEGDTVQIICNTGYRLQNNENNISCVERGWSTPPKCRSTDTSCVNPPTVQNAHILSRQMSKYPSGERVRYECRSPYEMFGDEEVMCLNGNWTEPPQCKDSTGKCGPPPPIDNGDITSFPLSVYAPASSVEYQCQNLYQLEGNKRITCRNGQWSEPPKCLHPCVISREIMENYNIALRWTAKQKLYLRTGESAEFVCKRGYRLSSRSHTLRTTCWDGKLEYPTCAKR

SEQ ID NO: 62 - DNA, 2334 bp, synthetic construct
  misc_feature 1..2334: note = nucleic acid sequence encoding PEDF-furin-P2A-CFHR1
  source 1..2334: mol_type = other DNA
atgcgccgcctggtgctgctgctgtgcatcggcgccctgctgggccacgtgttctgccagaaccccgccagcccccccgaggagggcagccccgaccccgacagcaccggcgccctggtggaggaggaggaccccttcttcaaggtgcccgtgaacaagctggccgccgccgtgagcaacttcggctacgacctgtaccgcgtgcgcagcagcaccagccccaccaccaacgtgctgctgagccccctgagcgtggccaccgccctgagcgccctgagcctgggcgccgagcagcgcaccgagagcatcatccaccgcgccctgtactacgacctgatcagcagccccgacatccacggcacctacaaggagctgctggacaccgtgaccgccccccagaagaacctgaagagcgccagccgcatcgtgttcgagaagaagctgcgcatcaagagcagcttcgtggcccccctggagaagagctacggcacccgcccccgcgtgctgaccggcaacccccgcctggacctgcaggagatcaacaactgggtgcaggcccagatgaagggcaagctggcccgcagcaccaaggagatccccgacgagatcagcatcctgctgctgggcgtggcccacttcaagggccagtgggtgaccaagttcgacagccgcaagaccagcctggaggacttctacctggacgaggagcgcaccgtgcgcgtgcccatgatgagcgaccccaaggccgtgctgcgctacggcctggacagcgacctgagctgcaagatcgcccagctgcccctgaccggcagcatgagcatcatcttcttcctgcccctgaaggtgacccagaacctgaccctgatcgaggagagcctgaccagcgagttcatccacgacatcgaccgcgagctgaagaccgtgcaggccgtgctgaccgtgcccaagctgaagctgagctacgagggcgaggtgaccaagagcctgcaggagatgaagctgcagagcctgttcgacagccccgacttcagcaagatcaccggcaagcccatcaagctgacccaggtggagcaccgcgccggcttcgagtggaacgaggacggcgccggcaccacccccagccccggcctgcagcccgcccacctgaccttccccctggactaccacctgaaccagcccttcatcttcgtgctgcgcgacaccgacaccggcgccctgctgttcatcggcaagatcctggacccccgcggcccccgccgcagcaagcgcagcggcagcggcgccaccaacttcagcctgctgaagcaggccggcgacgtggaggagaaccccggccccatgcgccgcttcctgaccgtgatcagcttcctgctgtacttcggctgcgccttcgccgaggccaccttctgcgacttccccaagatcaaccacggcatcctgtacgacgaggagaagtacaagcccttcagccaggtgcccaccggcgaggtgttctactacagctgcgagtacaacttcgtgagccccagcaagagcttctggacccgcatcacctgcaccgaggagggctggagccccacccccaagtgcctgcgcctgtgcttcttccccttcgtggagaacggccacagcgagagcagcggccagacccacctggagggcgacaccgtgcagatcatctgcaacaccggctaccgcctgcagaacaacgagaacaacatcagctgcgtggagcgcggctggagcaccccccccaagtgccgcagcaccgacaccagctgcgtgaacccccccaccgtgcagaacgcccacatcctgagccgccagatgagcaagtaccccagcggcgagcgcgtgcgctacgagtgccgcagcccctacgagatgttcggcgacgaggaggtgatgtgcctgaacggcaactggaccgagcccccccagtgcaaggacagcaccggcaagtgcggcccccccccccccatcgacaacggcgacatcaccagcttccccctgagcgtgtacgcccccgccagcagcgtggagtaccagtgccagaacctgtaccagctggagggcaacaagcgcatcacctgccgcaacggccagtggagcgagccccccaagtgcctgcacccctgcgtgatcagccgcgagatcatggagaactacaacatcgccctgcgctggaccgccaagcagaagctgtacctgcgcaccggcgagagcgccgagttcgtgtgcaagcgcggctaccgcctgagcagccgcagccacaccctgcgcaccacctgctgggacggcaagctggagtaccccacctgcgccaagcgctaa

SEQ ID NO: 63 - protein, 774 aa, synthetic construct
  REGION 1..774: note = CFHR1-furin-P2A- PEDF
MRRFLTVISFLLYFGCAFAEATFCDFPKINHGILYDEEKYKPFSQVPTGEVFYYSCEYNFVSPSKSFWTRITCTEEGWSPTPKCLRLCFFPFVENGHSESSGQTHLEGDTVQIICNTGYRLQNNENNISCVERGWSTPPKCRSTDTSCVNPPTVQNAHILSRQMSKYPSGERVRYECRSPYEMFGDEEVMCLNGNWTEPPQCKDSTGKCGPPPPIDNGDITSFPLSVYAPASSVEYQCQNLYQLEGNKRITCRNGQWSEPPKCLHPCVISREIMENYNIALRWTAKQKLYLRTGESAEFVCKRGYRLSSRSHTLRTTCWDGKLEYPTCAKRSKRSGSATNFSLLKQAGDVEENPGPMRRLVLLLCIGALLGHVFCQNPASPPEEGSPDPDSTGALVEEEDPFFKVPVNKLAAAVSNFGYDLYRVRSSTSPTTNVLLSPLSVATALSALSLGAEQRTESIIHRALYYDLISSPDIHGTYKELLDTVTAPQKNLKSASRIVFEKKLRIKSSFVAPLEKSYGTRPRVLTGNPRLDLQEINNWVQAQMKGKLARSTKEIPDEISILLLGVAHFKGQWVTKFDSRKTSLEDFYLDEERTVRVPMMSDPKAVLRYGLDSDLSCKIAQLPLTGSMSIIFFLPLKVTQNLTLIEESLTSEFIHDIDRELKTVQAVLTVPKLKLSYEGEVTKSLQEMKLQSLFDSPDFSKITGKPIKLTQVEHRAGFEWNEDGAGTTPSPGLQPAHLTFPLDYHLNQPFIFVLRDTDTGALLFIGKILDPRGP

SEQ ID NO: 64 - DNA, 2325 bp, synthetic construct
  misc_feature 1..2325: note = nucleic acid sequence encoding CFHR1-furin-P2A- PEDF
  source 1..2325: mol_type = other DNA
atgcgccgcctgctgaccttcatcagcatcctggccctggtgggcgccttcgccgaggccaccttctgcgacttccccaagatcaaccacggcatcctgtacgacgaggagaagtacaagcccttcagccaggtgcccaccggcgaggtgttctactacagctgcgagtacaacttcgtgagccccagcaagagcttctggacccgcatcacctgcaccgaggagggctggagccccacccccaagtgcctgcgcctgtgcttcttccccttcgtggagaacggccacagcgagagcagcggccagacccacctggagggcgacaccgtgcagatcatctgcaacaccggctaccgcctgcagaacaacgagaacaacatcagctgcgtggagcgcggctggagcaccccccccaagtgccgcagcaccgacaccagctgcgtgaacccccccaccgtgcagaacgcccacatcctgagccgccagatgagcaagtaccccagcggcgagcgcgtgcgctacgagtgccgcagcccctacgagatgttcggcgacgaggaggtgatgtgcctgaacggcaactggaccgagcccccccagtgcaaggacagcaccggcaagtgcggcccccccccccccatcgacaacggcgacatcaccagcttccccctgagcgtgtacgcccccgccagcagcgtggagtaccagtgccagaacctgtaccagctggagggcaacaagcgcatcacctgccgcaacggccagtggagcgagccccccaagtgcctgcacccctgcgtgatcagccgcgagatcatggagaactacaacatcgccctgcgctggaccgccaagcagaagctgtacctgcgcaccggcgagagcgccgagttcgtgtgcaagcgcggctaccgcctgagcagccgcagccacaccctgcgcaccacctgctgggacggcaagctggagtaccccacctgcgccaagcgcagcaagcgcagcggcagcggcgccaccaacttcagcctgctgaagcaggccggcgacgtggaggagaaccccggccccatgcgccgcctggtgctgctgctgtgcatcggcgccctgctgggccacgtgttctgccagaaccccgccagcccccccgaggagggcagccccgaccccgacagcaccggcgccctggtggaggaggaggaccccttcttcaaggtgcccgtgaacaagctggccgccgccgtgagcaacttcggctacgacctgtaccgcgtgcgcagcagcaccagccccaccaccaacgtgctgctgagccccctgagcgtggccaccgccctgagcgccctgagcctgggcgccgagcagcgcaccgagagcatcatccaccgcgccctgtactacgacctgatcagcagccccgacatccacggcacctacaaggagctgctggacaccgtgaccgccccccagaagaacctgaagagcgccagccgcatcgtgttcgagaagaagctgcgcatcaagagcagcttcgtggcccccctggagaagagctacggcacccgcccccgcgtgctgaccggcaacccccgcctggacctgcaggagatcaacaactgggtgcaggcccagatgaagggcaagctggcccgcagcaccaaggagatccccgacgagatcagcatcctgctgctgggcgtggcccacttcaagggccagtgggtgaccaagttcgacagccgcaagaccagcctggaggacttctacctggacgaggagcgcaccgtgcgcgtgcccatgatgagcgaccccaaggccgtgctgcgctacggcctggacagcgacctgagctgcaagatcgcccagctgcccctgaccggcagcatgagcatcatcttcttcctgcccctgaaggtgacccagaacctgaccctgatcgaggagagcctgaccagcgagttcatccacgacatcgaccgcgagctgaagaccgtgcaggccgtgctgaccgtgcccaagctgaagctgagctacgagggcgaggtgaccaagagcctgcaggagatgaagctgcagagcctgttcgacagccccgacttcagcaagatcaccggcaagcccatcaagctgacccaggtggagcaccgcgccggcttcgagtggaacgaggacggcgccggcaccacccccagccccggcctgcagcccgcccacctgaccttccccctggactaccacctgaaccagcccttcatcttcgtgctgcgcgacaccgacaccggcgccctgctgttcatcggcaagatcctggacccccgcggcccctaa

SEQ ID NO: 65 - protein, 709 aa, synthetic construct
  REGION 1..709: note = PEDF-furin-P2A-anti-Bb SCVF
MRRLVLLLCIGALLGHSSCQNPASPPEEGSPDPDSTGALVEEEDPFFKVPVNKLAAAVSNFGYDLYRVRSSTSPTTNVLLSPLSVATALSALSLGAEQRTESIIHRALYYDLISSPDIHGTYKELLDTVTAPQKNLKSASRIVFEKKLRIKSSFVAPLEKSYGTRPRVLTGNPRLDLQEINNWVQAQMKGKLARSTKEIPDEISILLLGVAHFKGQWVTKFDSRKTSLEDFYLDEERTVRVPMMSDPKAVLRYGLDSDLSCKIAQLPLTGSMSIIFFLPLKVTQNLTLIEESLTSEFIHDIDRELKTVQAVLTVPKLKLSYEGEVTKSLQEMKLQSLFDSPDFSKITGKPIKLTQVEHRAGFEWNEDGAGTTPSPGLQPAHLTFPLDYHLNQPFIFVLRDTDTGALLFIGKILDPRGPRVRRGSGATNFSLLKQAGDVEENPGPMRRLLILALVGAAVADVQITQSPSYLAASPGETITINCRASKSISKYLAWYQDKPGKTNKLLIYSGSTLQSGIPSRFSGSGSGTDFTLTISSLEPEDFAMYYCQQHDEYPWTFGGGTKLEIKRGGGGGSGGGGSGGGGSGGGGSQVQLQQSGAELAKPGASVRMSCKASGYTFTNYWIHWVKQRPGQGLEWIGYINPNTGYNDYNQKFKDKATLTADKSSSTVYMQLSSLTSEDSAVYYCARGGQLGLRRAMDYWGQGTSVTVSS

SEQ ID NO: 66 - DNA, 2130 bp, synthetic construct
  misc_feature 1..2130: note = nucleic acid sequence encoding PEDF-furin-P2A-anti-Bb SCVF
  source 1..2130: mol_type = other DNA
atgcgccgcctggtgctgctgctgtgcatcggcgccctgctgggccacagcagctgccagaaccccgccagcccccccgaggagggcagccccgaccccgacagcaccggcgccctggtggaggaggaggaccccttcttcaaggtgcccgtgaacaagctggccgccgccgtgagcaacttcggctacgacctgtaccgcgtgcgcagcagcaccagccccaccaccaacgtgctgctgagccccctgagcgtggccaccgccctgagcgccctgagcctgggcgccgagcagcgcaccgagagcatcatccaccgcgccctgtactacgacctgatcagcagccccgacatccacggcacctacaaggagctgctggacaccgtgaccgccccccagaagaacctgaagagcgccagccgcatcgtgttcgagaagaagctgcgcatcaagagcagcttcgtggcccccctggagaagagctacggcacccgcccccgcgtgctgaccggcaacccccgcctggacctgcaggagatcaacaactgggtgcaggcccagatgaagggcaagctggcccgcagcaccaaggagatccccgacgagatcagcatcctgctgctgggcgtggcccacttcaagggccagtgggtgaccaagttcgacagccgcaagaccagcctggaggacttctacctggacgaggagcgcaccgtgcgcgtgcccatgatgagcgaccccaaggccgtgctgcgctacggcctggacagcgacctgagctgcaagatcgcccagctgcccctgaccggcagcatgagcatcatcttcttcctgcccctgaaggtgacccagaacctgaccctgatcgaggagagcctgaccagcgagttcatccacgacatcgaccgcgagctgaagaccgtgcaggccgtgctgaccgtgcccaagctgaagctgagctacgagggcgaggtgaccaagagcctgcaggagatgaagctgcagagcctgttcgacagccccgacttcagcaagatcaccggcaagcccatcaagctgacccaggtggagcaccgcgccggcttcgagtggaacgaggacggcgccggcaccacccccagccccggcctgcagcccgcccacctgaccttccccctggactaccacctgaaccagcccttcatcttcgtgctgcgcgacaccgacaccggcgccctgctgttcatcggcaagatcctggacccccgcggcccccgcgtgcgccgcggcagcggcgccaccaacttcagcctgctgaagcaggccggcgacgtggaggagaaccccggccccatgcgccgcctgctgatcctggccctggtgggcgccgccgtggccgacgtccagatcacccagagccccagctacctggccgccagccccggcgagaccatcaccatcaactgccgcgccagcaagagcatcagcaagtacctggcctggtaccaggacaagcccggcaagaccaacaagctgctgatctacagcggcagcaccctgcagagcggcatccccagccgcttcagcggcagcggcagcggcaccgacttcaccctgaccatcagcagcctggagcccgaggacttcgccatgtactactgccagcagcacgacgagtacccctggaccttcggcggcggcaccaagctggagatcaagcgcggcggcggcggcggcagcggcggcggcggcagcggcggcggcggcagcggcggcggcggcagccaggtgcagctgcagcagagcggcgccgagctggccaagcccggcgccagcgtgcgcatgagctgcaaggccagcggctacaccttcaccaactactggatccactgggtgaagcagcgccccggccagggcctggagtggatcggctacatcaaccccaacaccggctacaacgactacaaccagaagttcaaggacaaggccaccctgaccgccgacaagagcagcagcaccgtgtacatgcagctgagcagcctgaccagcgaggacagcgccgtgtactactgcgcccgcggcggccagctgggcctgcgccgcgccatggactactggggccagggcaccagcgtgaccgtgagcagctga

SEQ ID NO: 67 - protein, 711 aa, synthetic construct
  REGION 1..711: note = PEDF-furin-P2A-anti-Bb SCVF
MRRLVLLLCIGALLGHSSCQNPASPPEEGSPDPDSTGALVEEEDPFFKVPVNKLAAAVSNFGYDLYRVRSSTSPTTNVLLSPLSVATALSALSLGAEQRTESIIHRALYYDLISSPDIHGTYKELLDTVTAPQKNLKSASRIVFEKKLRIKSSFVAPLEKSYGTRPRVLTGNPRLDLQEINNWVQAQMKGKLARSTKEIPDEISILLLGVAHFKGQWVTKFDSRKTSLEDFYLDEERTVRVPMMSDPKAVLRYGLDSDLSCKIAQLPLTGSMSIIFFLPLKVTQNLTLIEESLTSEFIHDIDRELKTVQAVLTVPKLKLSYEGEVTKSLQEMKLQSLFDSPDFSKITGKPIKLTQVEHRAGFEWNEDGAGTTPSPGLQPAHLTFPLDYHLNQPFIFVLRDTDTGALLFIGKILDPRGPRRSKRSGSGATNFSLLKQAGDVEENPGPMRRLLILALVGAAVADVQITQSPSYLAASPGETITINCRASKSISKYLAWYQDKPGKTNKLLIYSGSTLQSGIPSRFSGSGSGTDFTLTISSLEPEDFAMYYCQQHDEYPWTFGGGTKLEIKRGGGGGSGGGGSGGGGSGGGGSQVQLQQSGAELAKPGASVRMSCKASGYTFTNYWIHWVKQRPGQGLEWIGYINPNTGYNDYNQKFKDKATLTADKSSSTVYMQLSSLTSEDSAVYYCARGGQLGLRRAMDYWGQGTSVTVSS

SEQ ID NO: 68 - DNA, 2136 bp, synthetic construct
  misc_feature 1..2136: note = nucleic acid sequence encoding PEDF-furin-P2A-anti-Bb SCVF
  source 1..2136: mol_type = other DNA
atgcgccgcctggtgctgctgctgtgcatcggcgccctgctgggccacagcagctgccagaaccccgccagcccccccgaggagggcagccccgaccccgacagcaccggcgccctggtggaggaggaggaccccttcttcaaggtgcccgtgaacaagctggccgccgccgtgagcaacttcggctacgacctgtaccgcgtgcgcagcagcaccagccccaccaccaacgtgctgctgagccccctgagcgtggccaccgccctgagcgccctgagcctgggcgccgagcagcgcaccgagagcatcatccaccgcgccctgtactacgacctgatcagcagccccgacatccacggcacctacaaggagctgctggacaccgtgaccgccccccagaagaacctgaagagcgccagccgcatcgtgttcgagaagaagctgcgcatcaagagcagcttcgtggcccccctggagaagagctacggcacccgcccccgcgtgctgaccggcaacccccgcctggacctgcaggagatcaacaactgggtgcaggcccagatgaagggcaagctggcccgcagcaccaaggagatccccgacgagatcagcatcctgctgctgggcgtggcccacttcaagggccagtgggtgaccaagttcgacagccgcaagaccagcctggaggacttctacctggacgaggagcgcaccgtgcgcgtgcccatgatgagcgaccccaaggccgtgctgcgctacggcctggacagcgacctgagctgcaagatcgcccagctgcccctgaccggcagcatgagcatcatcttcttcctgcccctgaaggtgacccagaacctgaccctgatcgaggagagcctgaccagcgagttcatccacgacatcgaccgcgagctgaagaccgtgcaggccgtgctgaccgtgcccaagctgaagctgagctacgagggcgaggtgaccaagagcctgcaggagatgaagctgcagagcctgttcgacagccccgacttcagcaagatcaccggcaagcccatcaagctgacccaggtggagcaccgcgccggcttcgagtggaacgaggacggcgccggcaccacccccagccccggcctgcagcccgcccacctgaccttccccctggactaccacctgaaccagcccttcatcttcgtgctgcgcgacaccgacaccggcgccctgctgttcatcggcaagatcctggacccccgcggcccccgccgcagcaagcgcagcggcagcggcgccaccaacttcagcctgctgaagcaggccggcgacgtggaggagaaccccggccccatgcgccgcctgctgatcctggccctggtgggcgccgccgtggccgacgtccagatcacccagagccccagctacctggccgccagccccggcgagaccatcaccatcaactgccgcgccagcaagagcatcagcaagtacctggcctggtaccaggacaagcccggcaagaccaacaagctgctgatctacagcggcagcaccctgcagagcggcatccccagccgcttcagcggcagcggcagcggcaccgacttcaccctgaccatcagcagcctggagcccgaggacttcgccatgtactactgccagcagcacgacgagtacccctggaccttcggcggcggcaccaagctggagatcaagcgcggcggcggcggcggcagcggcggcggcggcagcggcggcggcggcagcggcggcggcggcagccaggtgcagctgcagcagagcggcgccgagctggccaagcccggcgccagcgtgcgcatgagctgcaaggccagcggctacaccttcaccaactactggatccactgggtgaagcagcgccccggccagggcctggagtggatcggctacatcaaccccaacaccggctacaacgactacaaccagaagttcaaggacaaggccaccctgaccgccgacaagagcagcagcaccgtgtacatgcagctgagcagcctgaccagcgaggacagcgccgtgtactactgcgcccgcggcggccagctgggcctgcgccgcgccatggactactggggccagggcaccagcgtgaccgtgagcagctga

SEQ ID NO: 69 - protein, 775 aa, synthetic construct
  REGION 1..775: note = PEDF-furin-P2A-sCD46
MRRLVLLLCIGALLGHVFCQNPASPPEEGSPDPDSTGALVEEEDPFFKVPVNKLAAAVSNFGYDLYRVRSSTSPTTNVLLSPLSVATALSALSLGAEQRTESIIHRALYYDLISSPDIHGTYKELLDTVTAPQKNLKSASRIVFEKKLRIKSSFVAPLEKSYGTRPRVLTGNPRLDLQEINNWVQAQMKGKLARSTKEIPDEISILLLGVAHFKGQWVTKFDSRKTSLEDFYLDEERTVRVPMMSDPKAVLRYGLDSDLSCKIAQLPLTGSMSIIFFLPLKVTQNLTLIEESLTSEFIHDIDRELKTVQAVLTVPKLKLSYEGEVTKSLQEMKLQSLFDSPDFSKITGKPIKLTQVEHRAGFEWNEDGAGTTPSPGLQPAHLTFPLDYHLNQPFIFVLRDTDTGALLFIGKILDPRGPRRSKRSGSGATNFSLLKQAGDVEENPGPMRRFLTVISFLLYFGCAFACEEPPTFEAMELIGKPKPYYEIGERVDYKCKKGYFYIPPLATHTICDRNHTWLPVSDDACYRETCPYIRDPLNGQAVPANGTYEFGYQMHFICNEGYYLIGEEILYCELKGSVAIWSGKPPICEKVLCTPPPKIKNGKHTFSEVEVFEYLDAVTYSCDPAPGPDPFSLIGESTIYCGDNSVWSRAAPECKVVKCRFPVVENGKQISGFGKKFYYKATVMFECDKGFYLDGSDTIVCDSNSTWDPPVPKCLKVLPPSSTKPPALSHSVSTSSTTKSPASSASGPRPTYKPPVSNYPGYPKPEEGILDSLDV

SEQ ID NO: 70 - DNA, 2328 bp, synthetic construct
  misc_feature 1..2328: note = nucleic acid sequence encoding PEDF-furin-P2A-sCD46
  source 1..2328: mol_type = other DNA
atgcgccgcctggtgctgctgctgtgcatcggcgccctgctgggccacgtgttctgccagaaccccgccagcccccccgaggagggcagccccgaccccgacagcaccggcgccctggtggaggaggaggaccccttcttcaaggtgcccgtgaacaagctggccgccgccgtgagcaacttcggctacgacctgtaccgcgtgcgcagcagcaccagccccaccaccaacgtgctgctgagccccctgagcgtggccaccgccctgagcgccctgagcctgggcgccgagcagcgcaccgagagcatcatccaccgcgccctgtactacgacctgatcagcagccccgacatccacggcacctacaaggagctgctggacaccgtgaccgccccccagaagaacctgaagagcgccagccgcatcgtgttcgagaagaagctgcgcatcaagagcagcttcgtggcccccctggagaagagctacggcacccgcccccgcgtgctgaccggcaacccccgcctggacctgcaggagatcaacaactgggtgcaggcccagatgaagggcaagctggcccgcagcaccaaggagatccccgacgagatcagcatcctgctgctgggcgtggcccacttcaagggccagtgggtgaccaagttcgacagccgcaagaccagcctggaggacttctacctggacgaggagcgcaccgtgcgcgtgcccatgatgagcgaccccaaggccgtgctgcgctacggcctggacagcgacctgagctgcaagatcgcccagctgcccctgaccggcagcatgagcatcatcttcttcctgcccctgaaggtgacccagaacctgaccctgatcgaggagagcctgaccagcgagttcatccacgacatcgaccgcgagctgaagaccgtgcaggccgtgctgaccgtgcccaagctgaagctgagctacgagggcgaggtgaccaagagcctgcaggagatgaagctgcagagcctgttcgacagccccgacttcagcaagatcaccggcaagcccatcaagctgacccaggtggagcaccgcgccggcttcgagtggaacgaggacggcgccggcaccacccccagccccggcctgcagcccgcccacctgaccttccccctggactaccacctgaaccagcccttcatcttcgtgctgcgcgacaccgacaccggcgccctgctgttcatcggcaagatcctggacccccgcggcccccgccgcagcaagcgcagcggcagcggcgccaccaacttcagcctgctgaagcaggccggcgacgtggaggagaaccccggccccatgcgccgcttcctgaccgtgatcagcttcctgctgtacttcggctgcgccttcgcctgcgaggagccccccaccttcgaggccatggagctgatcggcaagcccaagccctactacgagatcggcgagcgcgtggactacaagtgcaagaagggctacttctacatcccccccctggccacccacaccatctgcgaccgcaaccacacctggctgcccgtgagcgacgacgcctgctaccgcgagacctgcccctacatccgcgaccccctgaacggccaggccgtgcccgccaacggcacctacgagttcggctaccagatgcacttcatctgcaacgagggctactacctgatcggcgaggagatcctgtactgcgagctgaagggcagcgtggccatctggagcggcaagccccccatctgcgagaaggtgctgtgcacccccccccccaagatcaagaacggcaagcacaccttcagcgaggtggaggtgttcgagtacctggacgccgtgacctacagctgcgaccccgcccccggccccgaccccttcagcctgatcggcgagagcaccatctactgcggcgacaacagcgtgtggagccgcgccgcccccgagtgcaaggtggtgaagtgccgcttccccgtggtggagaacggcaagcagatcagcggcttcggcaagaagttctactacaaggccaccgtgatgttcgagtgcgacaagggcttctacctggacggcagcgacaccatcgtgtgcgacagcaacagcacctgggacccccccgtgcccaagtgcctgaaggtgctgccccccagcagcaccaagccccccgccctgagccacagcgtgagcaccagcagcaccaccaagagccccgccagcagcgccagcggcccccgccccacctacaagccccccgtgagcaactaccccggctaccccaagcccgaggagggcatcctggacagcctggacgtgtaa

SEQ ID NO: 71 - protein, 775 aa, synthetic construct
  REGION 1..775: note = sCD46-furin-P2A- PEDF
MRRFLTVISFLLYFGCAFACEEPPTFEAMELIGKPKPYYEIGERVDYKCKKGYFYIPPLATHTICDRNHTWLPVSDDACYRETCPYIRDPLNGQAVPANGTYEFGYQMHFICNEGYYLIGEEILYCELKGSVAIWSGKPPICEKVLCTPPPKIKNGKHTFSEVEVFEYLDAVTYSCDPAPGPDPFSLIGESTIYCGDNSVWSRAAPECKVVKCRFPVVENGKQISGFGKKFYYKATVMFECDKGFYLDGSDTIVCDSNSTWDPPVPKCLKVLPPSSTKPPALSHSVSTSSTTKSPASSASGPRPTYKPPVSNYPGYPKPEEGILDSLDVRRSKRSGSGATNFSLLKQAGDVEENPGPMRRLVLLLCIGALLGHVFCQNPASPPEEGSPDPDSTGALVEEEDPFFKVPVNKLAAAVSNFGYDLYRVRSSTSPTTNVLLSPLSVATALSALSLGAEQRTESIIHRALYYDLISSPDIHGTYKELLDTVTAPQKNLKSASRIVFEKKLRIKSSFVAPLEKSYGTRPRVLTGNPRLDLQEINNWVQAQMKGKLARSTKEIPDEISILLLGVAHFKGQWVTKFDSRKTSLEDFYLDEERTVRVPMMSDPKAVLRYGLDSDLSCKIAQLPLTGSMSIIFFLPLKVTQNLTLIEESLTSEFIHDIDRELKTVQAVLTVPKLKLSYEGEVTKSLQEMKLQSLFDSPDFSKITGKPIKLTQVEHRAGFEWNEDGAGTTPSPGLQPAHLTFPLDYHLNQPFIFVLRDTDTGALLFIGKILDPRGP

SEQ ID NO: 72 - DNA, 2328 bp, synthetic construct
  misc_feature 1..2328: note = nucleic acid sequence encoding sCD46-furin-P2A- PEDF
  source 1..2328: mol_type = other DNA
atgcgccgcttcctgaccgtgatcagcttcctgctgtacttcggctgcgccttcgcctgcgaggagccccccaccttcgaggccatggagctgatcggcaagcccaagccctactacgagatcggcgagcgcgtggactacaagtgcaagaagggctacttctacatcccccccctggccacccacaccatctgcgaccgcaaccacacctggctgcccgtgagcgacgacgcctgctaccgcgagacctgcccctacatccgcgaccccctgaacggccaggccgtgcccgccaacggcacctacgagttcggctaccagatgcacttcatctgcaacgagggctactacctgatcggcgaggagatcctgtactgcgagctgaagggcagcgtggccatctggagcggcaagccccccatctgcgagaaggtgctgtgcacccccccccccaagatcaagaacggcaagcacaccttcagcgaggtggaggtgttcgagtacctggacgccgtgacctacagctgcgaccccgcccccggccccgaccccttcagcctgatcggcgagagcaccatctactgcggcgacaacagcgtgtggagccgcgccgcccccgagtgcaaggtggtgaagtgccgcttccccgtggtggagaacggcaagcagatcagcggcttcggcaagaagttctactacaaggccaccgtgatgttcgagtgcgacaagggcttctacctggacggcagcgacaccatcgtgtgcgacagcaacagcacctgggacccccccgtgcccaagtgcctgaaggtgctgccccccagcagcaccaagccccccgccctgagccacagcgtgagcaccagcagcaccaccaagagccccgccagcagcgccagcggcccccgccccacctacaagccccccgtgagcaactaccccggctaccccaagcccgaggagggcatcctggacagcctggacgtgcgccgcagcaagcgcagcggcagcggcgccaccaacttcagcctgctgaagcaggccggcgacgtggaggagaaccccggccccatgcgccgcctggtgctgctgctgtgcatcggcgccctgctgggccacgtgttctgccagaaccccgccagcccccccgaggagggcagccccgaccccgacagcaccggcgccctggtggaggaggaggaccccttcttcaaggtgcccgtgaacaagctggccgccgccgtgagcaacttcggctacgacctgtaccgcgtgcgcagcagcaccagccccaccaccaacgtgctgctgagccccctgagcgtggccaccgccctgagcgccctgagcctgggcgccgagcagcgcaccgagagcatcatccaccgcgccctgtactacgacctgatcagcagccccgacatccacggcacctacaaggagctgctggacaccgtgaccgccccccagaagaacctgaagagcgccagccgcatcgtgttcgagaagaagctgcgcatcaagagcagcttcgtggcccccctggagaagagctacggcacccgcccccgcgtgctgaccggcaacccccgcctggacctgcaggagatcaacaactgggtgcaggcccagatgaagggcaagctggcccgcagcaccaaggagatccccgacgagatcagcatcctgctgctgggcgtggcccacttcaagggccagtgggtgaccaagttcgacagccgcaagaccagcctggaggacttctacctggacgaggagcgcaccgtgcgcgtgcccatgatgagcgaccccaaggccgtgctgcgctacggcctggacagcgacctgagctgcaagatcgcccagctgcccctgaccggcagcatgagcatcatcttcttcctgcccctgaaggtgacccagaacctgaccctgatcgaggagagcctgaccagcgagttcatccacgacatcgaccgcgagctgaagaccgtgcaggccgtgctgaccgtgcccaagctgaagctgagctacgagggcgaggtgaccaagagcctgcaggagatgaagctgcagagcctgttcgacagccccgacttcagcaagatcaccggcaagcccatcaagctgacccaggtggagcaccgcgccggcttcgagtggaacgaggacggcgccggcaccacccccagccccggcctgcagcccgcccacctgaccttccccctggactaccacctgaaccagcccttcatcttcgtgctgcgcgacaccgacaccggcgccctgctgttcatcggcaagatcctggacccccgcggcccctaa

SEQ ID NO: 73 - DNA, 4146 bp, synthetic construct
  misc_feature 1..4146: note = recombinant vector known as IKC0121V
  source 1..4146: mol_type = other DNA
cgcgctcgctcgctcactgaggccgcccgggcaaagcccgggcgtcgggcgacctttggtcgcccggcctcagtgagcgagcgagcgcgcagagagggagtggccaactccatcactaggggttccttgtagttaatgattaacccgccatgctacttatctacgtagccatgctctagacatggctcgacagatcgagctccaccgggtaccctagttattaatagtaatcaattacggggtcattagttcatagcccatatatggagttccgcgttacataacttacggtaaatggcccgcctggctgaccgcccaacgacccccgcccattgacgtcaataatgacgtatgttcccatagtaacgccaatagggactttccattgacgtcaatgggtggactatttacggtaaactgcccacttggcagtacatcaagtgtatcatatgccaagtacgccccctattgacgtcaatgacggtaaatggcccgcctggcattatgcccagtacatgaccttatgggactttcctacttggcagtacatctacgtattagtcatcgctattaccatggtcgaggtgagccccacgttctgcttcactctccccatctcccccccctccccacccccaattttgtatttatttattttttaattattttgtgcagcgatgggggcggggggggggggggggcgcgcgccaggcggggcggggcggggcgaggggcggggcggggcgaggcggagaggtgcggcggcagccaatcagagcggcgcgctccgaaagtttccttttatggcgaggcggcggcggcggcggccctataaaaagcgaagcgcgcggcgggcgggagtcgctgcgacgctgccttcgccccgtgccccgctccgccgccgcctcgcgccgcccgccccggctctgactgaccgcgttactcccacaggtgagcgggcgggacggcccttctcctccgggctgtaattagcgcttggtttaatgacggcttgtttcttttctgtggctgcgtgaaagccttgaggggctccgggaggctagagcctctgctaaccatgttcatgccttcttctttttcctacagctcctgggcaacgtgctggttattgtgctgtctcatcattttggcaaagaattcgcgactcgacccgctagcgccaccatgcgccgcctggtgctgctgctgtgcatcggcgccctgctgggccacgtgttctgccagaaccccgccagcccccccgaggagggcagccccgaccccgacagcaccggcgccctggtggaggaggaggaccccttcttcaaggtgcccgtgaacaagctggccgccgccgtgagcaacttcggctacgacctgtaccgcgtgcgcagcagcaccagccccaccaccaacgtgctgctgagccccctgagcgtggccaccgccctgagcgccctgagcctgggcgccgagcagcgcaccgagagcatcatccaccgcgccctgtactacgacctgatcagcagccccgacatccacggcacctacaaggagctgctggacaccgtgaccgccccccagaagaacctgaagagcgccagccgcatcgtgttcgagaagaagctgcgcatcaagagcagcttcgtggcccccctggagaagagctacggcacccgcccccgcgtgctgaccggcaacccccgcctggacctgcaggagatcaacaactgggtgcaggcccagatgaagggcaagctggcccgcagcaccaaggagatccccgacgagatcagcatcctgctgctgggcgtggcccacttcaagggccagtgggtgaccaagttcgacagccgcaagaccagcctggaggacttctacctggacgaggagcgcaccgtgcgcgtgcccatgatgagcgaccccaaggccgtgctgcgctacggcctggacagcgacctgagctgcaagatcgcccagctgcccctgaccggcagcatgagcatcatcttcttcctgcccctgaaggtgacccagaacctgaccctgatcgaggagagcctgaccagcgagttcatccacgacatcgaccgcgagctgaagaccgtgcaggccgtgctgaccgtgcccaagctgaagctgagctacgagggcgaggtgaccaagagcctgcaggagatgaagctgcagagcctgttcgacagccccgacttcagcaagatcaccggcaagcccatcaagctgacccaggtggagcaccgcgccggcttcgagtggaacgaggacggcgccggcaccacccccagccccggcctgcagcccgcccacctgaccttccccctggactaccacctgaaccagcccttcatcttcgtgctgcgcgacaccgacaccggcgccctgctgttcatcggcaagatcctggacccccgcggcccccgccgcagcaagcgcagcggcagcggcgccaccaacttcagcctgctgaagcaggccggcgacgtggaggagaaccccggccccatgcgccgcctgctgaccttcatcagcatcctggccctggtgggcgccttcgccgacatccagatgacccagagccccagcagcctgagcgccagcgtgggcgaccgcgtgaccatcacctgccgcgccagccaggacgtaagcaccgccgtggcctggtaccagcagaagcccggcaaggcccccaagctgctgatctacagcgccagcttcctgtacagcggcgtgcccagccgcttcagcggcagcggcagcggcaccgacttcaccctgaccatcagcagcctgcagcccgaggacttcgccacctactactgccagcagagctacgccaccctgcccaccttcgagcagggcaccaaggtggagatcaagcgcggcggcggcggcggcagcggcggcggcggcagcggcggcggcggcagcggcggcggcggcagcgaggtgcagctggtggagagcggcggcggcctggtgcagcccggcggcagcctgcgcctgagctgcgccgccagcggcttcagcttcaccagcagcagcgtgagccccggcaagggcctggagtgggtgggcctgatctacccctacaacggcttcaactactacgccgacagcgtgaagggccgcttcaccatcagcgccgacaccagcctgcagatgaacagcctgcgcgccgaggacaccgccgtgtactactgcgcccgcaacgccctgtacggcagcggcggctactacgccatggactactggggccagggcaccctggtgaccgtgagcagctgatatactactagtacgcggccgcaccggtgtacaatcaacctctggattacaaaatttgtgaaagattgactggtattcttaactatgttgctccttttacgctatgtggatacgctgctttaatgcctttgtatcatgctattgcttcccgtatggctttcattttctcctccttgtataaatcctggttagttcttgccacggcggaactcatcgccgcctgccttgcccgctgctggacaggggctcggctgttgggcactgacaattccgtggtgtgaattcgagctaggtacagcttatcgataccgtcgacagcagacatgataagatacattgatgagtttggacaaaccacaactagaatgcagtgaaaaaaatgctttatttgtgaaatttgtgatgctattgctttatttgtaaccattataagctgcaataaacaagttaacaacaacaattgcattcattttatgtttcaggttcagggggaggtgtgggaggttttttaaagcaagtaaaacctctacaaatgtggtatgctcgagggcatgcaacaacaacaattgcattcattttatgtttcaggttcagggggagatgtgggaggttttttaaagcaagtaaaacctctacaaatgtggtaaaatccgataaggactagagcatggctacgtagataagtagcatggcgggttaatcattaactacaaggaacccctagtgatggagttggccactccctctctgcgcgctcgctcgctcactgaggccgggcgaccaaaggtcgcccgacgcccgggctttgcccgggcggcctcagtgagcgagcgagcgcgc

SEQ ID NO: 74 - protein, 8 aa, synthetic construct
  REGION 1..8: note = gelatinase MMP-2 recognition sequence
GPQGIAGQ

SEQ ID NO: 75 - protein, 8 aa, synthetic construct
  REGION 1..8: note = gelatinase MMP-2 recognition sequence
GPLGIAGA

SEQ ID NO: 76 - protein, 8 aa, synthetic construct
  REGION 1..8: note = gelatinase MMP-2 recognition sequence
GPQGLLGQ

SEQ ID NO: 77 - protein, 8 aa, synthetic construct
  REGION 1..8: note = renin recognition sequence
HPFHLVYS

SEQ ID NO: 78 - protein, 9 aa, synthetic construct
  REGION 1..9: note = renin recognition sequence
HPFHLLVYS

SEQ ID NO: 79 - protein, 19 aa, synthetic construct
  REGION 1..19: note = endogenous signal peptide sequence
MQALVLLLCIGALLGHSSC

SEQ ID NO: 80 - protein, 426 aa, synthetic construct
  REGION 1..426: note = CFHL1
EDCNELPPRRNTEILTGSWSDQTYPEGTQAIYKCRPGYRSLGNVIMVCRKGEWVALNPLRKCQKRPCGHPGDTPFGTFTLTGGNVFEYGVKAVYTCNEGYQLLGEINYRECDTDGWTNDIPICEVVKCLPVTAPENGKIVSSAMEPDREYHFGQAVRFVCNSGYKIEGDEEMHCSDDGFWSKEKPKCVEISCKSPDVINGSPISQKIIYKENERFQYKCNMGYEYSERGDAVCTESGWRPLPSCEEKSCDNPYIPNGDYSPLRIKHRTGDEITYQCRNGFYPATRGNTAKCTSTGWIPAPRCTLKPCDYPDIKHGGLYHENMRRPYFPVAVGKYYSYYCDEHFETPSGSYWDHIHCTQDGWSPAVPCLRKCYFPYLENGYNQNYGRKFVQGKSIDVACHPGYALPKAQTTVTCMENGWSPTPRCIR

SEQ ID NO: 81 - DNA, 1278 bp, synthetic construct
  misc_feature 1..1278: note = nucleic acid sequence encoding CFHL1
  source 1..1278: mol_type = other DNA
gaggactgcaacgagctgcccccccgccgcaacaccgagatcctgaccggcagctggagcgaccagacctaccccgagggcacccaggccatctacaagtgccgccccggctaccgcagcctgggcaacgtgatcatggtgtgccgcaagggcgagtgggtggccctgaaccccctgcgcaagtgccagaagcgcccctgcggccaccccggcgacacccccttcggcaccttcaccctgaccggcggcaacgtgttcgagtacggcgtgaaggccgtgtacacctgcaacgagggctaccagctgctgggcgagatcaactaccgcgagtgcgacaccgacggctggaccaacgacatccccatctgcgaggtggtgaagtgcctgcccgtgaccgcccccgagaacggcaagatcgtgagcagcgccatggagcccgaccgcgagtaccacttcggccaggccgtgcgcttcgtgtgcaacagcggctacaagatcgagggcgacgaggagatgcactgcagcgacgacggcttctggagcaaggagaagcccaagtgcgtggagatcagctgcaagagccccgacgtgatcaacggcagccccatcagccagaagatcatctacaaggagaacgagcgcttccagtacaagtgcaacatgggctacgagtacagcgagcgcggcgacgccgtgtgcaccgagagcggctggcgccccctgcccagctgcgaggagaagagctgcgacaacccctacatccccaacggcgactacagccccctgcgcatcaagcaccgcaccggcgacgagatcacctaccagtgccgcaacggcttctaccccgccacccggggcaacaccgccaagtgcaccagcaccggctggatccccgccccccgctgcaccctgaagccctgcgactaccccgacatcaagcacggcggcctgtaccacgagaacatgcgccgcccctacttccccgtggccgtgggcaagtactacagctactactgcgacgagcacttcgagacccccagcggcagctactgggaccacatccactgcacccaggacggctggagccccgccgtgccctgcctgcgcaagtgctacttcccctacctggagaacggctacaaccagaactacggccgcaagttcgtgcagggcaagagcatcgacgtggcctgccaccccggctacgccctgcccaaggcccagaccaccgtgacctgcatggagaacggctggagccccaccccccgctgcatccgc

SEQ ID NO: 82 - protein, 252 aa, synthetic construct
  REGION 1..252: note = anti-C5 single chain variable fragment
DIQMTQSPSSLSASVGDRVTITCQASQSINNQLSWYQQKPGKAPKLLIYYASTLASGYPSRFSGSGSGTDFTLTISSLQPEDFATYYCQGSYYSGGWDYGFGQGTKVEIKRGGGGGSGGGSGGGGSGGGGSEVQLVESGGGLVQPGGSLRLSCAASGFSFSGRYWIQWVRQAPGKGLEWVASVWPGITGTNYANWAKGRFTISRDDSKNTLYLQMNSLRAEDTAVYYCAREPVAWGGGLDLWGQGTLVTVSS

SEQ ID NO: 83 - DNA, 759 bp, synthetic construct
  misc_feature 1..759: note = nucleic acid sequence encoding anti-C5 single chain variable fragment
  source 1..759: mol_type = other DNA
gacatccagatgacccagagccccagcagcctgagcgccagcgtgggcgaccgcgtgaccatcacctgccaggccagccagagcatcaacaaccagctgagctggtaccagcagaagcccggcaaggcccccaagctgctgatctactacgccagcaccctggccagcggctaccccagccgcttcagcggcagcggcagcggcaccgacttcaccctgaccatcagcagcctgcagcccgaggacttcgccacctactactgccagggcagctactacagcggcggctgggactacggcttcggccagggcaccaaggtggagatcaagcgcggcggcggcggcggcagcggcggcggcagcggcggcggcggcagcggcggcggcggcagcgaggtgcagctggtggagagcggcggcggcctggtgcagcccggcggcagcctgcgcctgagctgcgccgccagcggcttcagcttcagcggccgctactggatccagtgggtgcgccaggcccccggcaagggcctggagtgggtggccagcgtgtggcccggcatcaccggcaccaactacgccaactgggccaagggccgcttcaccatcagccgcgacgacagcaagaacaccctgtacctgcagatgaacagcctgcgcgccgaggacaccgccgtgtactactgcgcccgcgagcccgtggcctggggcggcggcctggacctgtggggccagggcaccctggtgaccgtgagcagctga

SEQ ID NO: 84 - DNA, 225 bp, synthetic construct
  misc_feature 1..225: note = nucliec acid sequence encoding bovine growth hormone
  source 1..225: mol_type = other DNA
ctgtgccttctagttgccagccatctgttgtttgcccctcccccgtgccttccttgaccctggaaggtgccactcccactgtcctttcctaataaaatgaggaaattgcatcgcattgtctgagtaggtgtcattctattctggggggtggggtggggcaggacagcaagggggaggattgggaagacaatagcaggcatgctggggatgcggtgggctctatgg

SEQ ID NO: 85 - protein, 711 aa, synthetic construct
  REGION 1..711: note = PEDF-furin-P2A-anti-C5 SCVF
MRRLVLLLCIGALLGHSSCQNPASPPEEGSPDPDSTGALVEEEDPFFKVPVNKLAAAVSNFGYDLYRVRSSTSPTTNVLLSPLSVATALSALSLGAEQRTESIIHRALYYDLISSPDIHGTYKELLDTVTAPQKNLKSASRIVFEKKLRIKSSFVAPLEKSYGTRPRVLTGNPRLDLQEINNWVQAQMKGKLARSTKEIPDEISILLLGVAHFKGQWVTKFDSRKTSLEDFYLDEERTVRVPMMSDPKAVLRYGLDSDLSCKIAQLPLTGSMSIIFFLPLKVTQNLTLIEESLTSEFIHDIDRELKTVQAVLTVPKLKLSYEGEVTKSLQEMKLQSLFDSPDFSKITGKPIKLTQVEHRAGFEWNEDGAGTTPSPGLQPAHLTFPLDYHLNQPFIFVLRDTDTGALLFIGKILDPRGPRVRRGSGATNFSLLKQAGDVEENPGPMRRLLILALVGAAVADIQMTQSPSSLSASVGDRVTITCQASQSINNQLSWYQQKPGKAPKLLIYYASTLASGYPSRFSGSGSGTDFTLTISSLQPEDFATYYCQGSYYSGGWDYGFGQGTKVEIKRGGGGGSGGGSGGGGSGGGGSEVQLVESGGGLVQPGGSLRLSCAASGFSFSGRYWIQWVRQAPGKGLEWVASVWPGITGTNYANWAKGRFTISRDDSKNTLYLQMNSLRAEDTAVYYCAREPVAWGGGLDLWGQGTLVTVSS

SEQ ID NO: 86 - DNA, 2136 bp, synthetic construct
  misc_feature 1..2136: note = nucleic acid sequence encoding PEDF-furin-P2A-anti-C5 SCVF
  source 1..2136: mol_type = other DNA
atgcgccgcctggtgctgctgctgtgcatcggcgccctgctgggccacagcagctgccagaaccccgccagcccccccgaggagggcagccccgaccccgacagcaccggcgccctggtggaggaggaggaccccttcttcaaggtgcccgtgaacaagctggccgccgccgtgagcaacttcggctacgacctgtaccgcgtgcgcagcagcaccagccccaccaccaacgtgctgctgagccccctgagcgtggccaccgccctgagcgccctgagcctgggcgccgagcagcgcaccgagagcatcatccaccgcgccctgtactacgacctgatcagcagccccgacatccacggcacctacaaggagctgctggacaccgtgaccgccccccagaagaacctgaagagcgccagccgcatcgtgttcgagaagaagctgcgcatcaagagcagcttcgtggcccccctggagaagagctacggcacccgcccccgcgtgctgaccggcaacccccgcctggacctgcaggagatcaacaactgggtgcaggcccagatgaagggcaagctggcccgcagcaccaaggagatccccgacgagatcagcatcctgctgctgggcgtggcccacttcaagggccagtgggtgaccaagttcgacagccgcaagaccagcctggaggacttctacctggacgaggagcgcaccgtgcgcgtgcccatgatgagcgaccccaaggccgtgctgcgctacggcctggacagcgacctgagctgcaagatcgcccagctgcccctgaccggcagcatgagcatcatcttcttcctgcccctgaaggtgacccagaacctgaccctgatcgaggagagcctgaccagcgagttcatccacgacatcgaccgcgagctgaagaccgtgcaggccgtgctgaccgtgcccaagctgaagctgagctacgagggcgaggtgaccaagagcctgcaggagatgaagctgcagagcctgttcgacagccccgacttcagcaagatcaccggcaagcccatcaagctgacccaggtggagcaccgcgccggcttcgagtggaacgaggacggcgccggcaccacccccagccccggcctgcagcccgcccacctgaccttccccctggactaccacctgaaccagcccttcatcttcgtgctgcgcgacaccgacaccggcgccctgctgttcatcggcaagatcctggacccccgcggcccccgcgtgcgccgcggcagcggcgccaccaacttcagcctgctgaagcaggccggcgacgtggaggagaaccccggccccatgcgccgcctgctgatcctggccctggtgggcgccgccgtggccgacatccagatgacccagagccccagcagcctgagcgccagcgtgggcgaccgcgtgaccatcacctgccaggccagccagagcatcaacaaccagctgagctggtaccagcagaagcccggcaaggcccccaagctgctgatctactacgccagcaccctggccagcggctaccccagccgcttcagcggcagcggcagcggcaccgacttcaccctgaccatcagcagcctgcagcccgaggacttcgccacctactactgccagggcagctactacagcggcggctgggactacggcttcggccagggcaccaaggtggagatcaagcgcggcggcggcggcggcagcggcggcggcagcggcggcggcggcagcggcggcggcggcagcgaggtgcagctggtggagagcggcggcggcctggtgcagcccggcggcagcctgcgcctgagctgcgccgccagcggcttcagcttcagcggccgctactggatccagtgggtgcgccaggcccccggcaagggcctggagtgggtggccagcgtgtggcccggcatcaccggcaccaactacgccaactgggccaagggccgcttcaccatcagccgcgacgacagcaagaacaccctgtacctgcagatgaacagcctgcgcgccgaggacaccgccgtgtactactgcgcccgcgagcccgtggcctggggcggcggcctggacctgtggggccagggcaccctggtgaccgtgagcagctga

SEQ ID NO: 87 - protein, 890 aa, synthetic construct
  REGION 1..890: note = PEDF-furin-P2A-CFHL1
MRRLVLLLCIGALLGHVFCQNPASPPEEGSPDPDSTGALVEEEDPFFKVPVNKLAAAVSNFGYDLYRVRSSTSPTTNVLLSPLSVATALSALSLGAEQRTESIIHRALYYDLISSPDIHGTYKELLDTVTAPQKNLKSASRIVFEKKLRIKSSFVAPLEKSYGTRPRVLTGNPRLDLQEINNWVQAQMKGKLARSTKEIPDEISILLLGVAHFKGQWVTKFDSRKTSLEDFYLDEERTVRVPMMSDPKAVLRYGLDSDLSCKIAQLPLTGSMSIIFFLPLKVTQNLTLIEESLTSEFIHDIDRELKTVQAVLTVPKLKLSYEGEVTKSLQEMKLQSLFDSPDFSKITGKPIKLTQVEHRAGFEWNEDGAGTTPSPGLQPAHLTFPLDYHLNQPFIFVLRDTDTGALLFIGKILDPRGPRRSKRSGSGATNFSLLKQAGDVEENPGPMRRLLTFISILALVGAFAEDCNELPPRRNTEILTGSWSDQTYPEGTQAIYKCRPGYRSLGNVIMVCRKGEWVALNPLRKCQKRPCGHPGDTPFGTFTLTGGNVFEYGVKAVYTCNEGYQLLGEINYRECDTDGWTNDIPICEVVKCLPVTAPENGKIVSSAMEPDREYHFGQAVRFVCNSGYKIEGDEEMHCSDDGFWSKEKPKCVEISCKSPDVINGSPISQKIIYKENERFQYKCNMGYEYSERGDAVCTESGWRPLPSCEEKSCDNPYIPNGDYSPLRIKHRTGDEITYQCRNGFYPATRGNTAKCTSTGWIPAPRCTLKPCDYPDIKHGGLYHENMRRPYFPVAVGKYYSYYCDEHFETPSGSYWDHIHCTQDGWSPAVPCLRKCYFPYLENGYNQNYGRKFVQGKSIDVACHPGYALPKAQTTVTCMENGWSPTPRCIR

SEQ ID NO: 88 - DNA, 2670 bp, synthetic construct
  misc_feature 1..2670: note = nucleic acid sequence encoding PEDF-furin-P2A-CFHL1
  source 1..2670: mol_type = other DNA
atgcgccgcctggtgctgctgctgtgcatcggcgccctgctgggccacgtgttctgccagaaccccgccagcccccccgaggagggcagccccgaccccgacagcaccggcgccctggtggaggaggaggaccccttcttcaaggtgcccgtgaacaagctggccgccgccgtgagcaacttcggctacgacctgtaccgcgtgcgcagcagcaccagccccaccaccaacgtgctgctgagccccctgagcgtggccaccgccctgagcgccctgagcctgggcgccgagcagcgcaccgagagcatcatccaccgcgccctgtactacgacctgatcagcagccccgacatccacggcacctacaaggagctgctggacaccgtgaccgccccccagaagaacctgaagagcgccagccgcatcgtgttcgagaagaagctgcgcatcaagagcagcttcgtggcccccctggagaagagctacggcacccgcccccgcgtgctgaccggcaacccccgcctggacctgcaggagatcaacaactgggtgcaggcccagatgaagggcaagctggcccgcagcaccaaggagatccccgacgagatcagcatcctgctgctgggcgtggcccacttcaagggccagtgggtgaccaagttcgacagccgcaagaccagcctggaggacttctacctggacgaggagcgcaccgtgcgcgtgcccatgatgagcgaccccaaggccgtgctgcgctacggcctggacagcgacctgagctgcaagatcgcccagctgcccctgaccggcagcatgagcatcatcttcttcctgcccctgaaggtgacccagaacctgaccctgatcgaggagagcctgaccagcgagttcatccacgacatcgaccgcgagctgaagaccgtgcaggccgtgctgaccgtgcccaagctgaagctgagctacgagggcgaggtgaccaagagcctgcaggagatgaagctgcagagcctgttcgacagccccgacttcagcaagatcaccggcaagcccatcaagctgacccaggtggagcaccgcgccggcttcgagtggaacgaggacggcgccggcaccacccccagccccggcctgcagcccgcccacctgaccttccccctggactaccacctgaaccagcccttcatcttcgtgctgcgcgacaccgacaccggcgccctgctgttcatcggcaagatcctggacccccgcggcccccgccgcagcaagcgcagcggcagcggcgccaccaacttcagcctgctgaagcaggccggcgacgtggaggagaaccccggccccatgcgccgcctgctgaccttcatcagcatcctggccctggtgggcgccttcgccgaggactgcaacgagctgcccccccgccgcaacaccgagatcctgaccggcagctggagcgaccagacctaccccgagggcacccaggccatctacaagtgccgccccggctaccgcagcctgggcaacgtgatcatggtgtgccgcaagggcgagtgggtggccctgaaccccctgcgcaagtgccagaagcgcccctgcggccaccccggcgacacccccttcggcaccttcaccctgaccggcggcaacgtgttcgagtacggcgtgaaggccgtgtacacctgcaacgagggctaccagctgctgggcgagatcaactaccgcgagtgcgacaccgacggctggaccaacgacatccccatctgcgaggtggtgaagtgcctgcccgtgaccgcccccgagaacggcaagatcgtgagcagcgccatggagcccgaccgcgagtaccacttcggccaggccgtgcgcttcgtgtgcaacagcggctacaagatcgagggcgacgaggagatgcactgcagcgacgacggcttctggagcaaggagaagcccaagtgcgtggagatcagctgcaagagccccgacgtgatcaacggcagccccatcagccagaagatcatctacaaggagaacgagcgcttccagtacaagtgcaacatgggctacgagtacagcgagcgcggcgacgccgtgtgcaccgagagcggctggcgccccctgcccagctgcgaggagaagagctgcgacaacccctacatccccaacggcgactacagccccctgcgcatcaagcaccgcaccggcgacgagatcacctaccagtgccgcaacggcttctaccccgccacccggggcaacaccgccaagtgcaccagcaccggctggatccccgccccccgctgcaccctgaagccctgcgactaccccgacatcaagcacggcggcctgtaccacgagaacatgcgccgcccctacttccccgtggccgtgggcaagtactacagctactactgcgacgagcacttcgagacccccagcggcagctactgggaccacatccactgcacccaggacggctggagccccgccgtgccctgcctgcgcaagtgctacttcccctacctggagaacggctacaaccagaactacggccgcaagttcgtgcagggcaagagcatcgacgtggcctgccaccccggctacgccctgcccaaggcccagaccaccgtgacctgcatggagaacggctggagccccaccccccgctgcatccgc

SEQ ID NO: 89 - protein, 890 aa, synthetic construct
  REGION 1..890: note = CFHL1-furin-P2A-PEDF
MRRLLTFISILALVGAFAEDCNELPPRRNTEILTGSWSDQTYPEGTQAIYKCRPGYRSLGNVIMVCRKGEWVALNPLRKCQKRPCGHPGDTPFGTFTLTGGNVFEYGVKAVYTCNEGYQLLGEINYRECDTDGWTNDIPICEVVKCLPVTAPENGKIVSSAMEPDREYHFGQAVRFVCNSGYKIEGDEEMHCSDDGFWSKEKPKCVEISCKSPDVINGSPISQKIIYKENERFQYKCNMGYEYSERGDAVCTESGWRPLPSCEEKSCDNPYIPNGDYSPLRIKHRTGDEITYQCRNGFYPATRGNTAKCTSTGWIPAPRCTLKPCDYPDIKHGGLYHENMRRPYFPVAVGKYYSYYCDEHFETPSGSYWDHIHCTQDGWSPAVPCLRKCYFPYLENGYNQNYGRKFVQGKSIDVACHPGYALPKAQTTVTCMENGWSPTPRCIRRRSKRSGSGATNFSLLKQAGDVEENPGPMRRLVLLLCIGALLGHVFCQNPASPPEEGSPDPDSTGALVEEEDPFFKVPVNKLAAAVSNFGYDLYRVRSSTSPTTNVLLSPLSVATALSALSLGAEQRTESIIHRALYYDLISSPDIHGTYKELLDTVTAPQKNLKSASRIVFEKKLRIKSSFVAPLEKSYGTRPRVLTGNPRLDLQEINNWVQAQMKGKLARSTKEIPDEISILLLGVAHFKGQWVTKFDSRKTSLEDFYLDEERTVRVPMMSDPKAVLRYGLDSDLSCKIAQLPLTGSMSIIFFLPLKVTQNLTLIEESLTSEFIHDIDRELKTVQAVLTVPKLKLSYEGEVTKSLQEMKLQSLFDSPDFSKITGKPIKLTQVEHRAGFEWNEDGAGTTPSPGLQPAHLTFPLDYHLNQPFIFVLRDTDTGALLFIGKILDPRGP

SEQ ID NO: 90 - DNA, 2670 bp, synthetic construct
  misc_feature 1..2670: note = nucleic acid sequence encoding CFHL1-furin-P2A-PEDF
  source 1..2670: mol_type = other DNA
atgcgccgcctgctgaccttcatcagcatcctggccctggtgggcgccttcgccgaggactgcaacgagctgcccccccgccgcaacaccgagatcctgaccggcagctggagcgaccagacctaccccgagggcacccaggccatctacaagtgccgccccggctaccgcagcctgggcaacgtgatcatggtgtgccgcaagggcgagtgggtggccctgaaccccctgcgcaagtgccagaagcgcccctgcggccaccccggcgacacccccttcggcaccttcaccctgaccggcggcaacgtgttcgagtacggcgtgaaggccgtgtacacctgcaacgagggctaccagctgctgggcgagatcaactaccgcgagtgcgacaccgacggctggaccaacgacatccccatctgcgaggtggtgaagtgcctgcccgtgaccgcccccgagaacggcaagatcgtgagcagcgccatggagcccgaccgcgagtaccacttcggccaggccgtgcgcttcgtgtgcaacagcggctacaagatcgagggcgacgaggagatgcactgcagcgacgacggcttctggagcaaggagaagcccaagtgcgtggagatcagctgcaagagccccgacgtgatcaacggcagccccatcagccagaagatcatctacaaggagaacgagcgcttccagtacaagtgcaacatgggctacgagtacagcgagcgcggcgacgccgtgtgcaccgagagcggctggcgccccctgcccagctgcgaggagaagagctgcgacaacccctacatccccaacggcgactacagccccctgcgcatcaagcaccgcaccggcgacgagatcacctaccagtgccgcaacggcttctaccccgccacccggggcaacaccgccaagtgcaccagcaccggctggatccccgccccccgctgcaccctgaagccctgcgactaccccgacatcaagcacggcggcctgtaccacgagaacatgcgccgcccctacttccccgtggccgtgggcaagtactacagctactactgcgacgagcacttcgagacccccagcggcagctactgggaccacatccactgcacccaggacggctggagccccgccgtgccctgcctgcgcaagtgctacttcccctacctggagaacggctacaaccagaactacggccgcaagttcgtgcagggcaagagcatcgacgtggcctgccaccccggctacgccctgcccaaggcccagaccaccgtgacctgcatggagaacggctggagccccaccccccgctgcatccgccgccgcagcaagcgcagcggcagcggcgccaccaacttcagcctgctgaagcaggccggcgacgtggaggagaaccccggccccatgcgccgcctggtgctgctgctgtgcatcggcgccctgctgggccacgtgttctgccagaaccccgccagcccccccgaggagggcagccccgaccccgacagcaccggcgccctggtggaggaggaggaccccttcttcaaggtgcccgtgaacaagctggccgccgccgtgagcaacttcggctacgacctgtaccgcgtgcgcagcagcaccagccccaccaccaacgtgctgctgagccccctgagcgtggccaccgccctgagcgccctgagcctgggcgccgagcagcgcaccgagagcatcatccaccgcgccctgtactacgacctgatcagcagccccgacatccacggcacctacaaggagctgctggacaccgtgaccgccccccagaagaacctgaagagcgccagccgcatcgtgttcgagaagaagctgcgcatcaagagcagcttcgtggcccccctggagaagagctacggcacccgcccccgcgtgctgaccggcaacccccgcctggacctgcaggagatcaacaactgggtgcaggcccagatgaagggcaagctggcccgcagcaccaaggagatccccgacgagatcagcatcctgctgctgggcgtggcccacttcaagggccagtgggtgaccaagttcgacagccgcaagaccagcctggaggacttctacctggacgaggagcgcaccgtgcgcgtgcccatgatgagcgaccccaaggccgtgctgcgctacggcctggacagcgacctgagctgcaagatcgcccagctgcccctgaccggcagcatgagcatcatcttcttcctgcccctgaaggtgacccagaacctgaccctgatcgaggagagcctgaccagcgagttcatccacgacatcgaccgcgagctgaagaccgtgcaggccgtgctgaccgtgcccaagctgaagctgagctacgagggcgaggtgaccaagagcctgcaggagatgaagctgcagagcctgttcgacagccccgacttcagcaagatcaccggcaagcccatcaagctgacccaggtggagcaccgcgccggcttcgagtggaacgaggacggcgccggcaccacccccagccccggcctgcagcccgcccacctgaccttccccctggactaccacctgaaccagcccttcatcttcgtgctgcgcgacaccgacaccggcgccctgctgttcatcggcaagatcctggacccccgcggcccc